European Patent Specification EP 3 927 168 B1, published September 3, 2025. Title: ENGINEERED PESTICIDAL PROTEINS. Applicant: Syngenta Participations AG Chae, Hyunsook Sarah. The sequence listing filed with the application follows.

SEQUENCE LISTING (35 sequences)

SEQ ID NO: 1 - protein, 715 aa, Artificial sequence
  BT-0022 sequence assembled from Bacillus genome mining
MKSKNQNMHQSLSNNATVDKNFTGSLENNTNTELQNFNHEGIEPFVSVSTIQTGIGIAGKILGNLGVPFAGQVASLYSFILGELWPKGKSQWEIFMEHVEELINQKISTYARNKALADLKGLGDALAVYHESLESWIKNRNNTRTRSVVKSQYITLELMFVQSLPSFAVSGEEVPLLPIYAQAANLHLLLLRDASIFGKEWGLSDSEISTFYNRQVERTSDYSDHCTKWFDTGLNRLKGSNAEIWVKYNQFRRDMTLMVLDLVALFQSYDTHMYPIKTTAQLTREVYTNAIGTVHPHPSFTSTTWYNNNAPSFSAIEAAVIRSPHLLDFLEQVTIYSLLSRWSNTQYMNMWGGHKLEFRTIGGTLNTSTQGSTNTSINPVTLPFTSRDIYRTESLAGLNLFLTQPVNGVPRVDFHWKFVTHPIASDNFYYPGYAGIGTQLQDSENELPPETTGQPNYESYSHRLSHIGLISASHVKALVYSWTHRSADRTNTIHSDSITQIPLVKAHTLQSGTTVVKGPGFTGGDILRRTSGGPFAFSNVNLDWNLSQRYRARIRYASTTNLRMYVTIAGERIFAGQFNKTMNTGDPLTFQSFSYATIDTAFTFPTKASSLTVGADTFSSGNEVYVDRFELIPVTATLEAVTDLERAQKAVHELFTSTNPGGLKTDVAKDHYTNTISKSVQSVFRCRCSERTRIYRWGYPSKKEYWYIWGYTSKY

SEQ ID NO: 2 - protein, 1131 aa, Artificial sequence
  BT-0002 sequence assembled from Bacillus genome mining
MEINNQKQCIPYNCLSNPEEVLLDGERILPDIDPLEVSLSLLQFLLNNFVPGGGFISGLVDKIWGALRPSEWDLFLAQIERLIDQRIEATVRAKAIAELEGLGRSYQLYGEAFKEWEKTPDNTAARSRVTERFRIIDAQIEANIPSFRVSGFEVPLLLVYTQAANLHLALLRDSVVFGERWGLTTTNVNDIYNRQVNRIGEYSNHCVDTYNTELERLGFRSIAQWRIYNQFRRELTLTVLDIVALFPNYDSRLYPIQTFSQLTREIVTSPVSEFYYGVINSGNINGTLTEQQIRRPHLMDFFNSMIMYTSDNRREHYWSGLEMTAYFTGFAGAQVSFPLVGTRGESAPPLTVRSVNDGIYRILSAPFYSAPFLGTIVLGSRGEKFDFALNNISPPPSTIYRHPGTVDSLVSIPPQDNSVPPHRGSSHRLSHVTMRASSPIFHWTHRSATTTNTINPNAIIQIPLVKAFNLHSGATVVRGPGFTGGDILRRTNTGTFADMRVNITGPLSQRYRVRIRYASTTDLQFFTRINGTSVNQGNFQRTMNRGDNLESGNFRTAGFSTPFSFSNAQSTFTLGTQAFSNQEVYIDRIEFVPAEVTFEAESDLERAQKAVNALFTSTNQLGLKTDVTDYQIDQVSNLVECLSDEFCLDEKRELSEKVKHAKRLSDKRNLLQDPNFTSINRQLDRGWRGSTDITIQGGNDVFKENYVTLPGTFDECYPTYLYQKIDESKLKAYTRYELRGYIEDSQDLEVYLIRYNAKHETVNVPGTGSLWPLSVESPIGRCGEPNRCVPHIEWNPDLDCSCRDGEKCAHHSHHFSLDIDVGCTDLNEDLGVWVIFKIKTQDGHARLGNLEFLEEKPLLGEALARVKRAEKKWRDKREQLQFETNIVYKEAKESVDALFVDSHYNRLQADTNITMIHAADKRVHRIREAYLPELSVIPGVNADIFEELEGLIFTAFSLYDARNIIKNGDFNNGLSCWNVKGHVDIQQNDHRSVLVVPEWESEVSQEVRVCPGRGYILRVTAYKEGYGEGCVTIHEIEDNTDELKFSNCIEEEVYPTDTGNDYTAHQGTTGCADACNSRNVGYEDGYEINTTASVNYKPTYEEEMYTDVRRDNHCEYDRGYGNHTPLPAGYV

SEQ ID NO: 3 - protein, 1174 aa, Bacillus thuringiensis
MENNIQNQCVPYNCLNNPEVEILNEERSTGRLPLDISLSLTRFLLSEFVPGVGVAFGLFDLIWGFITPSDWSLFLLQIEQLIEQRIETLERNRAITTLRGLADSYEIYIEALREWEANPNNAQLREDVRIRFANTDDALITAINNFTLTSFEIPLLSVYVQAANLHLSLLRDAVSFGQGWGLDIATVNNHYNRLINLIHRYTKHCLDTYNQGLENLRGTNTRQWARFNQFRRDLTLTVLDIVALFPNYDVRTYPIQTSSQLTREIYTSSVIEDSPVSANIPNGFNRAEFGVRPPHLMDFMNSLFVTAETVRSQTVWGGHLVSSRNTAGNRINFPSYGVFNPGGAIWIADEDPRPFYRTLSDPVFVRGGFGNPHYVLGLRGVAFQQTGTNHTRTFRNSGTIDSLDEIPPQDNSGAPWNDYSHVLNHVTFVRWPGEISGSDSWRAPMFSWTHRSATPTNTIDPERITQIPLVKAHTLQSGTTVVRGPGFTGGDILRRTSGGPFAYTIVNINGQLPQRYRARIRYASTTNLRIYVTVAGERIFAGQFNKTMDTGDPLTFQSFSYATINTAFTFPMSQSSFTVGADTFSSGNEVYIDRFELIPVTATFEAEYDLERAQKAVNALFTSINQIGIKTDVTDYHIDQVSNLVDCLSDEFCLDEKRELSEKVKHAKRLSDERNLLQDPNFKGINRQLDRGWRGSTDITIQRGDDVFKENYVTLPGTFDECYPTYLYQKIDESKLKPYTRYQLRGYIEDSQDLEIYLIRYNAKHETVNVLGTGSLWPLSVQSPIRKCGEPNRCAPHLEWNPDLDCSCRDGEKCAHHSHHFSLDIDVGCTDLNEDLDVWVIFKIKTQDGHARLGNLEFLEEKPLVGEALARVKRAEKKWRDKREKLELETNIVYKEAKESVDALFVNSQYDQLQADTNIAMIHAADKRVHRIREAYLPELSVIPGVNVDIFEELKGRIFTAFFLYDARNVIKNGDFNNGLSCWNVKGHVDVEEQNNHRSVLVVPEWEAEVSQEVRVCPGRGYILRVTAYKEGYGEGCVTIHEIENNTDELKFSNCVEEEVYPNNTVTCNDYTANQEEYGGAYTSRNRGYDETYGSNSSVPADYASVYEEKSYTDGRRDNPCESNRGYGDYTPLPAGYVTKELEYFPETDKVWIEIGETEGTFIVDSVELLLMEE

SEQ ID NO: 4 - protein, 1168 aa, Artificial Sequence
  Modified Bt toxin
MEINNQKQCIPYNCLSNPEEVLLDGERILPDIDPLEVSLSLLQFLLNNFVPGGGFISGLVDKIWGALRPSEWDLFLAQIERLIDQRIEATVRAKAIAELEGLGRSYQLYGEAFKEWEKTPDNTAARSRVTERFRIIDAQIEANIPSFRVSGFEVPLLLVYTQAANLHLALLRDSVVFGERWGLTTTNVNDIYNRQVNRIGEYSNHCVDTYNTELERLGFRSIAQWRIYNQFRRELTLTVLDIVALFPNYDSRLYPIQTFSQLTREIVTSPVSEFYYGVINSGNINGTLTEQQIRRPHLMDFFNSMIMYTSDNRREHYWSGLEMTAYFTGFAGAQVSFPLVGTRGESAPPLTVRSVNDGIYRILSAPFYSAPFLGTIVLGSRGEKFDFALNNISPPPSTIYRHPGTVDSLVSIPPQDNSVPPHRGSSHRLSHVTMRASSPIFHWTHRSATTTNTINPNAIIQIPLVKAHTLQSGTTVVKGPGFTGGDILRRTSGGPFAFSNVNLDWNLSQRYRARIRYASTTNLRMYVTIAGERIFAGQFNKTMNTGDPLTFQSFSYATIDTAFTFPTKASSLTVGADTFSSGNEVYVDRFELIPVTATFEAESDLERAQKAVNALFTSTNQLGLKTDVTDYQIDQVSNLVECLSDEFCLDEKRELSEKVKHAKRLSDKRNLLQDPNFTSINRQLDRGWRGSTDITIQGGNDVFKENYVTLPGTFDECYPTYLYQKIDESKLKAYTRYELRGYIEDSQDLEVYLIRYNAKHETVNVPGTGSLWPLSVESPIGRCGEPNRCVPHIEWNPDLDCSCRDGEKCAHHSHHFSLDIDVGCTDLNEDLGVWVIFKIKTQDGHARLGNLEFLEEKPLLGEALARVKRAEKKWRDKREQLQFETNIVYKEAKESVDALFVDSHYNRLQADTNITMIHAADKRVHRIREAYLPELSVIPGVNADIFEELEGLIFTAFSLYDARNIIKNGDFNNGLSCWNVKGHVDIQQNDHRSVLVVPEWESEVSQEVRVCPGRGYILRVTAYKEGYGEGCVTIHEIEDNTDELKFSNCIEEEVYPTDTGNDYTAHQGTTGCADACNSRNVGYEDGYEINTTASVNYKPTYEEEMYTDVRRDNHCEYDRGYGNHTPLPAGYVTKELEYFPETDTVWIEIGETEGTFIVDSVELLLMEE

SEQ ID NO: 5 - protein, 1168 aa, Artificial Sequence
  Modified Bt toxin
MEINNQKQCIPYNCLSNPEEVLLDGERILPDIDPLEVSLSLLQFLLNNFVPGGGFISGLVDKIWGALRPSEWDLFLAQIERLIDQRIEATVRAKAIAELEGLGRSYQLYGEAFKEWEKTPDNTAARSRVTERFRIIDAQIEANIPSFRVSGFEVPLLLVYTQAANLHLALLRDSVVFGERWGLTTTNVNDIYNRQVNRIGEYSNHCVDTYNTELERLGFRSIAQWRIYNQFRRELTLTVLDIVALFPNYDSRLYPIQTFSQLTREIVTSPVSEFYYGVINSGNINGTLTEQQIRRPHLMDFFNSMIMYTSDNRREHYWSGLEMTAYFTGFAGAQVSFPLVGTRGESAPPLTVRSVNDGIYRILSAPFYSAPFLGTIVLGSRGEKFDFALNNISPPPSTIYRHPGTVDSLVSIPPQDNSVPPHRGSSHRLSHVTMRASSPIFHWTHRSATTTNTIHSDSITQIPLVKAHTLQSGTTVVKGPGFTGGDILRRTSGGPFAFSNVNLDWNLSQRYRARIRYASTTNLRMYVTIAGERIFAGQFNKTMNTGDPLTFQSFSYATIDTAFTFPTKASSLTVGADTFSSGNEVYVDRFELIPVTATFEAESDLERAQKAVNALFTSTNQLGLKTDVTDYQIDQVSNLVECLSDEFCLDEKRELSEKVKHAKRLSDKRNLLQDPNFTSINRQLDRGWRGSTDITIQGGNDVFKENYVTLPGTFDECYPTYLYQKIDESKLKAYTRYELRGYIEDSQDLEVYLIRYNAKHETVNVPGTGSLWPLSVESPIGRCGEPNRCVPHIEWNPDLDCSCRDGEKCAHHSHHFSLDIDVGCTDLNEDLGVWVIFKIKTQDGHARLGNLEFLEEKPLLGEALARVKRAEKKWRDKREQLQFETNIVYKEAKESVDALFVDSHYNRLQADTNITMIHAADKRVHRIREAYLPELSVIPGVNADIFEELEGLIFTAFSLYDARNIIKNGDFNNGLSCWNVKGHVDIQQNDHRSVLVVPEWESEVSQEVRVCPGRGYILRVTAYKEGYGEGCVTIHEIEDNTDELKFSNCIEEEVYPTDTGNDYTAHQGTTGCADACNSRNVGYEDGYEINTTASVNYKPTYEEEMYTDVRRDNHCEYDRGYGNHTPLPAGYVTKELEYFPETDTVWIEIGETEGTFIVDSVELLLMEE

SEQ ID NO: 6 - protein, 1168 aa, Artificial Sequence
  Modified Bt toxin
MEINNQKQCIPYNCLSNPEEVLLDGERILPDIDPLEVSLSLLQFLLNNFVPGGGFISGLVDKIWGALRPSEWDLFLAQIERLIDQRIEATVRAKAIAELEGLGRSYQLYGEAFKEWEKTPDNTAARSRVTERFRIIDAQIEANIPSFRVSGFEVPLLLVYTQAANLHLALLRDSVVFGERWGLTTTNVNDIYNRQVNRIGEYSNHCVDTYNTELERLGFRSIAQWRIYNQFRRELTLTVLDIVALFPNYDSRLYPIQTFSQLTREIVTSPVSEFYYGVINSGNINGTLTEQQIRRPHLMDFFNSMIMYTSDNRREHYWSGLEMTAYFTGFAGAQVSFPLVGTRGESAPPLTVRSVNDGIYRILSAPFYSAPFLGTIVLGSRGEKFDFALNNISPPPSTIYRHPGTVDSLVSIPPQDNSVPPHRGSSHRLSHVTMRASSPIFHWTHRSADRTNTIHSDSITQIPLVKAHTLQSGTTVVKGPGFTGGDILRRTSGGPFAFSNVNLDWNLSQRYRARIRYASTTNLRMYVTIAGERIFAGQFNKTMNTGDPLTFQSFSYATIDTAFTFPTKASSLTVGADTFSSGNEVYVDRFELIPVTATFEAESDLERAQKAVNALFTSTNQLGLKTDVTDYQIDQVSNLVECLSDEFCLDEKRELSEKVKHAKRLSDKRNLLQDPNFTSINRQLDRGWRGSTDITIQGGNDVFKENYVTLPGTFDECYPTYLYQKIDESKLKAYTRYELRGYIEDSQDLEVYLIRYNAKHETVNVPGTGSLWPLSVESPIGRCGEPNRCVPHIEWNPDLDCSCRDGEKCAHHSHHFSLDIDVGCTDLNEDLGVWVIFKIKTQDGHARLGNLEFLEEKPLLGEALARVKRAEKKWRDKREQLQFETNIVYKEAKESVDALFVDSHYNRLQADTNITMIHAADKRVHRIREAYLPELSVIPGVNADIFEELEGLIFTAFSLYDARNIIKNGDFNNGLSCWNVKGHVDIQQNDHRSVLVVPEWESEVSQEVRVCPGRGYILRVTAYKEGYGEGCVTIHEIEDNTDELKFSNCIEEEVYPTDTGNDYTAHQGTTGCADACNSRNVGYEDGYEINTTASVNYKPTYEEEMYTDVRRDNHCEYDRGYGNHTPLPAGYVTKELEYFPETDTVWIEIGETEGTFIVDSVELLLMEE

SEQ ID NO: 7 - protein, 1168 aa, Artificial Sequence
  Modified Bt toxin
MEINNQKQCIPYNCLSNPEEVLLDGERILPDIDPLEVSLSLLQFLLNNFVPGGGFISGLVDKIWGALRPSEWDLFLAQIERLIDQRIEATVRAKAIAELEGLGRSYQLYGEAFKEWEKTPDNTAARSRVTERFRIIDAQIEANIPSFRVSGFEVPLLLVYTQAANLHLALLRDSVVFGERWGLTTTNVNDIYNRQVNRIGEYSNHCVDTYNTELERLGFRSIAQWRIYNQFRRELTLTVLDIVALFPNYDSRLYPIQTFSQLTREIVTSPVSEFYYGVINSGNINGTLTEQQIRRPHLMDFFNSMIMYTSDNRREHYWSGLEMTAYFTGFAGAQVSFPLVGTRGESAPPLTVRSVNDGIYRILSAPFYSAPFLGTIVLGSRGEKFDFALNNISPPPSTIYRHPGTVDSLVSIPPQDNSVPPHRGSSHRLSHVTMRASSPIFHWTHRSATTTNTINPNAIIQIPLVKAHTLQSGTTVVKGPGFTGGDILRRTSGGPFAFSNVNLDWNLSQRYRARIRYASTTNLRMYVTIAGERIFAGQFNKTMNTGDPLTFQSFSYATIDTAFTFPTKASSLTVGADTFSSGNEVYVDRFELIPVTATLEAVTDLERAQKAVNALFTSTNQLGLKTDVTDYQIDQVSNLVECLSDEFCLDEKRELSEKVKHAKRLSDKRNLLQDPNFTSINRQLDRGWRGSTDITIQGGNDVFKENYVTLPGTFDECYPTYLYQKIDESKLKAYTRYELRGYIEDSQDLEVYLIRYNAKHETVNVPGTGSLWPLSVESPIGRCGEPNRCVPHIEWNPDLDCSCRDGEKCAHHSHHFSLDIDVGCTDLNEDLGVWVIFKIKTQDGHARLGNLEFLEEKPLLGEALARVKRAEKKWRDKREQLQFETNIVYKEAKESVDALFVDSHYNRLQADTNITMIHAADKRVHRIREAYLPELSVIPGVNADIFEELEGLIFTAFSLYDARNIIKNGDFNNGLSCWNVKGHVDIQQNDHRSVLVVPEWESEVSQEVRVCPGRGYILRVTAYKEGYGEGCVTIHEIEDNTDELKFSNCIEEEVYPTDTGNDYTAHQGTTGCADACNSRNVGYEDGYEINTTASVNYKPTYEEEMYTDVRRDNHCEYDRGYGNHTPLPAGYVTKELEYFPETDTVWIEIGETEGTFIVDSVELLLMEE

SEQ ID NO: 8 - protein, 1168 aa, Artificial Sequence
  Modified Bt toxin
MEINNQKQCIPYNCLSNPEEVLLDGERILPDIDPLEVSLSLLQFLLNNFVPGGGFISGLVDKIWGALRPSEWDLFLAQIERLIDQRIEATVRAKAIAELEGLGRSYQLYGEAFKEWEKTPDNTAARSRVTERFRIIDAQIEANIPSFRVSGFEVPLLLVYTQAANLHLALLRDSVVFGERWGLTTTNVNDIYNRQVNRIGEYSNHCVDTYNTELERLGFRSIAQWRIYNQFRRELTLTVLDIVALFPNYDSRLYPIQTFSQLTREIVTSPVSEFYYGVINSGNINGTLTEQQIRRPHLMDFFNSMIMYTSDNRREHYWSGLEMTAYFTGFAGAQVSFPLVGTRGESAPPLTVRSVNDGIYRILSAPFYSAPFLGTIVLGSRGEKFDFALNNISPPPSTIYRHPGTVDSLVSIPPQDNSVPPHRGSSHRLSHVTMRASSPIFHWTHRSATTTNTIHSDSITQIPLVKAHTLQSGTTVVKGPGFTGGDILRRTSGGPFAFSNVNLDWNLSQRYRARIRYASTTNLRMYVTIAGERIFAGQFNKTMNTGDPLTFQSFSYATIDTAFTFPTKASSLTVGADTFSSGNEVYVDRFELIPVTATLEAVTDLERAQKAVNALFTSTNQLGLKTDVTDYQIDQVSNLVECLSDEFCLDEKRELSEKVKHAKRLSDKRNLLQDPNFTSINRQLDRGWRGSTDITIQGGNDVFKENYVTLPGTFDECYPTYLYQKIDESKLKAYTRYELRGYIEDSQDLEVYLIRYNAKHETVNVPGTGSLWPLSVESPIGRCGEPNRCVPHIEWNPDLDCSCRDGEKCAHHSHHFSLDIDVGCTDLNEDLGVWVIFKIKTQDGHARLGNLEFLEEKPLLGEALARVKRAEKKWRDKREQLQFETNIVYKEAKESVDALFVDSHYNRLQADTNITMIHAADKRVHRIREAYLPELSVIPGVNADIFEELEGLIFTAFSLYDARNIIKNGDFNNGLSCWNVKGHVDIQQNDHRSVLVVPEWESEVSQEVRVCPGRGYILRVTAYKEGYGEGCVTIHEIEDNTDELKFSNCIEEEVYPTDTGNDYTAHQGTTGCADACNSRNVGYEDGYEINTTASVNYKPTYEEEMYTDVRRDNHCEYDRGYGNHTPLPAGYVTKELEYFPETDTVWIEIGETEGTFIVDSVELLLMEE

SEQ ID NO: 9 - protein, 1168 aa, Artificial Sequence
  Modified Bt toxin
MEINNQKQCIPYNCLSNPEEVLLDGERILPDIDPLEVSLSLLQFLLNNFVPGGGFISGLVDKIWGALRPSEWDLFLAQIERLIDQRIEATVRAKAIAELEGLGRSYQLYGEAFKEWEKTPDNTAARSRVTERFRIIDAQIEANIPSFRVSGFEVPLLLVYTQAANLHLALLRDSVVFGERWGLTTTNVNDIYNRQVNRIGEYSNHCVDTYNTELERLGFRSIAQWRIYNQFRRELTLTVLDIVALFPNYDSRLYPIQTFSQLTREIVTSPVSEFYYGVINSGNINGTLTEQQIRRPHLMDFFNSMIMYTSDNRREHYWSGLEMTAYFTGFAGAQVSFPLVGTRGESAPPLTVRSVNDGIYRILSAPFYSAPFLGTIVLGSRGEKFDFALNNISPPPSTIYRHPGTVDSLVSIPPQDNSVPPHRGSSHRLSHVTMRASSPIFHWTHRSADRTNTIHSDSITQIPLVKAHTLQSGTTVVKGPGFTGGDILRRTSGGPFAFSNVNLDWNLSQRYRARIRYASTTNLRMYVTIAGERIFAGQFNKTMNTGDPLTFQSFSYATIDTAFTFPTKASSLTVGADTFSSGNEVYVDRFELIPVTATLEAVTDLERAQKAVNALFTSTNQLGLKTDVTDYQIDQVSNLVECLSDEFCLDEKRELSEKVKHAKRLSDKRNLLQDPNFTSINRQLDRGWRGSTDITIQGGNDVFKENYVTLPGTFDECYPTYLYQKIDESKLKAYTRYELRGYIEDSQDLEVYLIRYNAKHETVNVPGTGSLWPLSVESPIGRCGEPNRCVPHIEWNPDLDCSCRDGEKCAHHSHHFSLDIDVGCTDLNEDLGVWVIFKIKTQDGHARLGNLEFLEEKPLLGEALARVKRAEKKWRDKREQLQFETNIVYKEAKESVDALFVDSHYNRLQADTNITMIHAADKRVHRIREAYLPELSVIPGVNADIFEELEGLIFTAFSLYDARNIIKNGDFNNGLSCWNVKGHVDIQQNDHRSVLVVPEWESEVSQEVRVCPGRGYILRVTAYKEGYGEGCVTIHEIEDNTDELKFSNCIEEEVYPTDTGNDYTAHQGTTGCADACNSRNVGYEDGYEINTTASVNYKPTYEEEMYTDVRRDNHCEYDRGYGNHTPLPAGYVTKELEYFPETDTVWIEIGETEGTFIVDSVELLLMEE

SEQ ID NO: 10 - protein, 1168 aa, Artificial Sequence
  Modified Bt toxin
MEINNQKQCIPYNCLSNPEEVLLDGERILPDIDPLEVSLSLLQFLLNNFVPGGGFISGLVDKIWGALRPSEWDLFLAQIERLIDQRIEATVRAKAIAELEGLGRSYQLYGEAFKEWEKTPDNTAARSRVTERFRIIDAQIEANIPSFRVSGFEVPLLLVYTQAANLHLALLRDSVVFGERWGLTTTNVNDIYNRQVNRIGEYSNHCVDTYNTELERLGFRSIAQWRIYNQFRRELTLTVLDIVALFPNYDSRLYPIQTFSQLTREIVTSPVSEFYYGVINSGNINGTLTEQQIRRPHLMDFFNSMIMYTSDNRREHYWSGLEMTAYFTGFAGAQVSFPLVGTRGESAPPLTVRSVNDGIYRILSAPFYSAPFLGTIVLGSRGEKFDFALNNISPPPSTIYRHPGTVDSLVSIPPQDNSVPPHRGSSHRLSHVTMRASSPIFHWTHRSATTTNTIHSDSITQIPLVKAHTLQSGTTVVKGPGFTGGDILRRTSGGPFAFSNVNLDWNLSQRYRARIRYASTTNLRMYVTIAGERIFAGQFNKTMNTGDPLTFQSFSYATIDTAFTFPTKASSLTVGADTFSSGNEVYVDRFELIPVTATFEAEYDLERAQKAVNALFTSTNQLGLKTDVTDYQIDQVSNLVECLSDEFCLDEKRELSEKVKHAKRLSDKRNLLQDPNFTSINRQLDRGWRGSTDITIQGGNDVFKENYVTLPGTFDECYPTYLYQKIDESKLKAYTRYELRGYIEDSQDLEVYLIRYNAKHETVNVPGTGSLWPLSVESPIGRCGEPNRCVPHIEWNPDLDCSCRDGEKCAHHSHHFSLDIDVGCTDLNEDLGVWVIFKIKTQDGHARLGNLEFLEEKPLLGEALARVKRAEKKWRDKREQLQFETNIVYKEAKESVDALFVDSHYNRLQADTNITMIHAADKRVHRIREAYLPELSVIPGVNADIFEELEGLIFTAFSLYDARNIIKNGDFNNGLSCWNVKGHVDIQQNDHRSVLVVPEWESEVSQEVRVCPGRGYILRVTAYKEGYGEGCVTIHEIEDNTDELKFSNCIEEEVYPTDTGNDYTAHQGTTGCADACNSRNVGYEDGYEINTTASVNYKPTYEEEMYTDVRRDNHCEYDRGYGNHTPLPAGYVTKELEYFPETDTVWIEIGETEGTFIVDSVELLLMEE

SEQ ID NO: 11 - protein, 1168 aa, Artificial Sequence
  Modified Bt toxin
MEINNQKQCIPYNCLSNPEEVLLDGERILPDIDPLEVSLSLLQFLLNNFVPGGGFISGLVDKIWGALRPSEWDLFLAQIERLIDQRIEATVRAKAIAELEGLGRSYQLYGEAFKEWEKTPDNTAARSRVTERFRIIDAQIEANIPSFRVSGFEVPLLLVYTQAANLHLALLRDSVVFGERWGLTTTNVNDIYNRQVNRIGEYSNHCVDTYNTELERLGFRSIAQWRIYNQFRRELTLTVLDIVALFPNYDSRLYPIQTFSQLTREIVTSPVSEFYYGVINSGNINGTLTEQQIRRPHLMDFFNSMIMYTSDNRREHYWSGLEMTAYFTGFAGAQVSFPLVGTRGESAPPLTVRSVNDGIYRILSAPFYSAPFLGTIVLGSRGEKFDFALNNISPPPSTIYRHPGTVDSLVSIPPQDNSVPPHRGSSHRLSHVTMRASSPIFHWTHRSADRTNTIHSDSITQIPLVKAHTLQSGTTVVKGPGFTGGDILRRTSGGPFAFSNVNLDWNLSQRYRARIRYASTTNLRMYVTIAGERIFAGQFNKTMNTGDPLTFQSFSYATIDTAFTFPTKASSLTVGADTFSSGNEVYVDRFELIPVTATFEAEYDLERAQKAVNALFTSTNQLGLKTDVTDYQIDQVSNLVECLSDEFCLDEKRELSEKVKHAKRLSDKRNLLQDPNFTSINRQLDRGWRGSTDITIQGGNDVFKENYVTLPGTFDECYPTYLYQKIDESKLKAYTRYELRGYIEDSQDLEVYLIRYNAKHETVNVPGTGSLWPLSVESPIGRCGEPNRCVPHIEWNPDLDCSCRDGEKCAHHSHHFSLDIDVGCTDLNEDLGVWVIFKIKTQDGHARLGNLEFLEEKPLLGEALARVKRAEKKWRDKREQLQFETNIVYKEAKESVDALFVDSHYNRLQADTNITMIHAADKRVHRIREAYLPELSVIPGVNADIFEELEGLIFTAFSLYDARNIIKNGDFNNGLSCWNVKGHVDIQQNDHRSVLVVPEWESEVSQEVRVCPGRGYILRVTAYKEGYGEGCVTIHEIEDNTDELKFSNCIEEEVYPTDTGNDYTAHQGTTGCADACNSRNVGYEDGYEINTTASVNYKPTYEEEMYTDVRRDNHCEYDRGYGNHTPLPAGYVTKELEYFPETDTVWIEIGETEGTFIVDSVELLLMEE

SEQ ID NO: 12 - protein, 1168 aa, Artificial Sequence
  Modified Bt toxin
MEINNQKQCIPYNCLSNPEEVLLDGERILPDIDPLEVSLSLLQFLLNNFVPGGGFISGLVDKIWGALRPSEWDLFLAQIERLIDQRIEATVRAKAIAELEGLGRSYQLYGEAFKEWEKTPDNTAARSRVTERFRIIDAQIEANIPSFRVSGFEVPLLLVYTQAANLHLALLRDSVVFGERWGLTTTNVNDIYNRQVNRIGEYSNHCVDTYNTELERLGFRSIAQWRIYNQFRRELTLTVLDIVALFPNYDSRLYPIQTFSQLTREIVTSPVSEFYYGVINSGNINGTLTEQQIRRPHLMDFFNSMIMYTSDNRREHYWSGLEMTAYFTGFAGAQVSFPLVGTRGESAPPLTVRSVNDGIYRILSAPFYSAPFLGTIVLGSRGEKFDFALNNISPPPSTIYRHPGTVDSLVSIPPQDNSVPPHRGSSHRLSHVTMRASSPIFHWTHRSATTTNTINPNAIIQIPLVKAHTLQSGTTVVRGPGFTGGDILRRTSGGPFAYTIVNINGQLPQRYRARIRYASTTNLRIYVTVAGERIFAGQFNKTMDTGDPLTFQSFSYATINTAFTFPMSQSSFTVGADTFSSGNEVYIDRFELIPVTATFEAESDLERAQKAVNALFTSTNQLGLKTDVTDYQIDQVSNLVECLSDEFCLDEKRELSEKVKHAKRLSDKRNLLQDPNFTSINRQLDRGWRGSTDITIQGGNDVFKENYVTLPGTFDECYPTYLYQKIDESKLKAYTRYELRGYIEDSQDLEVYLIRYNAKHETVNVPGTGSLWPLSVESPIGRCGEPNRCVPHIEWNPDLDCSCRDGEKCAHHSHHFSLDIDVGCTDLNEDLGVWVIFKIKTQDGHARLGNLEFLEEKPLLGEALARVKRAEKKWRDKREQLQFETNIVYKEAKESVDALFVDSHYNRLQADTNITMIHAADKRVHRIREAYLPELSVIPGVNADIFEELEGLIFTAFSLYDARNIIKNGDFNNGLSCWNVKGHVDIQQNDHRSVLVVPEWESEVSQEVRVCPGRGYILRVTAYKEGYGEGCVTIHEIEDNTDELKFSNCIEEEVYPTDTGNDYTAHQGTTGCADACNSRNVGYEDGYEINTTASVNYKPTYEEEMYTDVRRDNHCEYDRGYGNHTPLPAGYVTKELEYFPETDTVWIEIGETEGTFIVDSVELLLMEE

SEQ ID NO: 13 - protein, 1168 aa, Artificial Sequence
  Modified Bt toxin
MEINNQKQCIPYNCLSNPEEVLLDGERILPDIDPLEVSLSLLQFLLNNFVPGGGFISGLVDKIWGALRPSEWDLFLAQIERLIDQRIEATVRAKAIAELEGLGRSYQLYGEAFKEWEKTPDNTAARSRVTERFRIIDAQIEANIPSFRVSGFEVPLLLVYTQAANLHLALLRDSVVFGERWGLTTTNVNDIYNRQVNRIGEYSNHCVDTYNTELERLGFRSIAQWRIYNQFRRELTLTVLDIVALFPNYDSRLYPIQTFSQLTREIVTSPVSEFYYGVINSGNINGTLTEQQIRRPHLMDFFNSMIMYTSDNRREHYWSGLEMTAYFTGFAGAQVSFPLVGTRGESAPPLTVRSVNDGIYRILSAPFYSAPFLGTIVLGSRGEKFDFALNNISPPPSTIYRHPGTVDSLVSIPPQDNSVPPHRGSSHRLSHVTMRASSPIFHWTHRSATTTNTIDPERITQIPLVKAHTLQSGTTVVRGPGFTGGDILRRTSGGPFAYTIVNINGQLPQRYRARIRYASTTNLRIYVTVAGERIFAGQFNKTMDTGDPLTFQSFSYATINTAFTFPMSQSSFTVGADTFSSGNEVYIDRFELIPVTATFEAESDLERAQKAVNALFTSTNQLGLKTDVTDYQIDQVSNLVECLSDEFCLDEKRELSEKVKHAKRLSDKRNLLQDPNFTSINRQLDRGWRGSTDITIQGGNDVFKENYVTLPGTFDECYPTYLYQKIDESKLKAYTRYELRGYIEDSQDLEVYLIRYNAKHETVNVPGTGSLWPLSVESPIGRCGEPNRCVPHIEWNPDLDCSCRDGEKCAHHSHHFSLDIDVGCTDLNEDLGVWVIFKIKTQDGHARLGNLEFLEEKPLLGEALARVKRAEKKWRDKREQLQFETNIVYKEAKESVDALFVDSHYNRLQADTNITMIHAADKRVHRIREAYLPELSVIPGVNADIFEELEGLIFTAFSLYDARNIIKNGDFNNGLSCWNVKGHVDIQQNDHRSVLVVPEWESEVSQEVRVCPGRGYILRVTAYKEGYGEGCVTIHEIEDNTDELKFSNCIEEEVYPTDTGNDYTAHQGTTGCADACNSRNVGYEDGYEINTTASVNYKPTYEEEMYTDVRRDNHCEYDRGYGNHTPLPAGYVTKELEYFPETDTVWIEIGETEGTFIVDSVELLLMEE

SEQ ID NO: 14 - protein, 1168 aa, Artificial Sequence
  Modified Bt toxin
MEINNQKQCIPYNCLSNPEEVLLDGERILPDIDPLEVSLSLLQFLLNNFVPGGGFISGLVDKIWGALRPSEWDLFLAQIERLIDQRIEATVRAKAIAELEGLGRSYQLYGEAFKEWEKTPDNTAARSRVTERFRIIDAQIEANIPSFRVSGFEVPLLLVYTQAANLHLALLRDSVVFGERWGLTTTNVNDIYNRQVNRIGEYSNHCVDTYNTELERLGFRSIAQWRIYNQFRRELTLTVLDIVALFPNYDSRLYPIQTFSQLTREIVTSPVSEFYYGVINSGNINGTLTEQQIRRPHLMDFFNSMIMYTSDNRREHYWSGLEMTAYFTGFAGAQVSFPLVGTRGESAPPLTVRSVNDGIYRILSAPFYSAPFLGTIVLGSRGEKFDFALNNISPPPSTIYRHPGTVDSLVSIPPQDNSVPPHRGSSHRLSHVTMRASSPIFHWTHRSATPTNTIDPERITQIPLVKAHTLQSGTTVVRGPGFTGGDILRRTSGGPFAYTIVNINGQLPQRYRARIRYASTTNLRIYVTVAGERIFAGQFNKTMDTGDPLTFQSFSYATINTAFTFPMSQSSFTVGADTFSSGNEVYIDRFELIPVTATFEAESDLERAQKAVNALFTSTNQLGLKTDVTDYQIDQVSNLVECLSDEFCLDEKRELSEKVKHAKRLSDKRNLLQDPNFTSINRQLDRGWRGSTDITIQGGNDVFKENYVTLPGTFDECYPTYLYQKIDESKLKAYTRYELRGYIEDSQDLEVYLIRYNAKHETVNVPGTGSLWPLSVESPIGRCGEPNRCVPHIEWNPDLDCSCRDGEKCAHHSHHFSLDIDVGCTDLNEDLGVWVIFKIKTQDGHARLGNLEFLEEKPLLGEALARVKRAEKKWRDKREQLQFETNIVYKEAKESVDALFVDSHYNRLQADTNITMIHAADKRVHRIREAYLPELSVIPGVNADIFEELEGLIFTAFSLYDARNIIKNGDFNNGLSCWNVKGHVDIQQNDHRSVLVVPEWESEVSQEVRVCPGRGYILRVTAYKEGYGEGCVTIHEIEDNTDELKFSNCIEEEVYPTDTGNDYTAHQGTTGCADACNSRNVGYEDGYEINTTASVNYKPTYEEEMYTDVRRDNHCEYDRGYGNHTPLPAGYVTKELEYFPETDTVWIEIGETEGTFIVDSVELLLMEE

SEQ ID NO: 15 - protein, 1168 aa, Artificial Sequence
  Modified Bt toxin
MEINNQKQCIPYNCLSNPEEVLLDGERILPDIDPLEVSLSLLQFLLNNFVPGGGFISGLVDKIWGALRPSEWDLFLAQIERLIDQRIEATVRAKAIAELEGLGRSYQLYGEAFKEWEKTPDNTAARSRVTERFRIIDAQIEANIPSFRVSGFEVPLLLVYTQAANLHLALLRDSVVFGERWGLTTTNVNDIYNRQVNRIGEYSNHCVDTYNTELERLGFRSIAQWRIYNQFRRELTLTVLDIVALFPNYDSRLYPIQTFSQLTREIVTSPVSEFYYGVINSGNINGTLTEQQIRRPHLMDFFNSMIMYTSDNRREHYWSGLEMTAYFTGFAGAQVSFPLVGTRGESAPPLTVRSVNDGIYRILSAPFYSAPFLGTIVLGSRGEKFDFALNNISPPPSTIYRHPGTVDSLVSIPPQDNSVPPHRGSSHRLSHVTMRASSPIFHWTHRSATTTNTINPNAIIQIPLVKAHTLQSGTTVVRGPGFTGGDILRRTSGGPFAYTIVNINGQLPQRYRARIRYASTTNLRIYVTVAGERIFAGQFNKTMDTGDPLTFQSFSYATINTAFTFPMSQSSFTVGADTFSSGNEVYIDRFELIPVTATFEAEYDLERAQKAVNALFTSTNQLGLKTDVTDYQIDQVSNLVECLSDEFCLDEKRELSEKVKHAKRLSDKRNLLQDPNFTSINRQLDRGWRGSTDITIQGGNDVFKENYVTLPGTFDECYPTYLYQKIDESKLKAYTRYELRGYIEDSQDLEVYLIRYNAKHETVNVPGTGSLWPLSVESPIGRCGEPNRCVPHIEWNPDLDCSCRDGEKCAHHSHHFSLDIDVGCTDLNEDLGVWVIFKIKTQDGHARLGNLEFLEEKPLLGEALARVKRAEKKWRDKREQLQFETNIVYKEAKESVDALFVDSHYNRLQADTNITMIHAADKRVHRIREAYLPELSVIPGVNADIFEELEGLIFTAFSLYDARNIIKNGDFNNGLSCWNVKGHVDIQQNDHRSVLVVPEWESEVSQEVRVCPGRGYILRVTAYKEGYGEGCVTIHEIEDNTDELKFSNCIEEEVYPTDTGNDYTAHQGTTGCADACNSRNVGYEDGYEINTTASVNYKPTYEEEMYTDVRRDNHCEYDRGYGNHTPLPAGYVTKELEYFPETDTVWIEIGETEGTFIVDSVELLLMEE

SEQ ID NO: 16 - protein, 1168 aa, Artificial Sequence
  Modified Bt toxin
MEINNQKQCIPYNCLSNPEEVLLDGERILPDIDPLEVSLSLLQFLLNNFVPGGGFISGLVDKIWGALRPSEWDLFLAQIERLIDQRIEATVRAKAIAELEGLGRSYQLYGEAFKEWEKTPDNTAARSRVTERFRIIDAQIEANIPSFRVSGFEVPLLLVYTQAANLHLALLRDSVVFGERWGLTTTNVNDIYNRQVNRIGEYSNHCVDTYNTELERLGFRSIAQWRIYNQFRRELTLTVLDIVALFPNYDSRLYPIQTFSQLTREIVTSPVSEFYYGVINSGNINGTLTEQQIRRPHLMDFFNSMIMYTSDNRREHYWSGLEMTAYFTGFAGAQVSFPLVGTRGESAPPLTVRSVNDGIYRILSAPFYSAPFLGTIVLGSRGEKFDFALNNISPPPSTIYRHPGTVDSLVSIPPQDNSVPPHRGSSHRLSHVTMRASSPIFHWTHRSATTTNTIDPERITQIPLVKAHTLQSGTTVVRGPGFTGGDILRRTSGGPFAYTIVNINGQLPQRYRARIRYASTTNLRIYVTVAGERIFAGQFNKTMDTGDPLTFQSFSYATINTAFTFPMSQSSFTVGADTFSSGNEVYIDRFELIPVTATFEAEYDLERAQKAVNALFTSTNQLGLKTDVTDYQIDQVSNLVECLSDEFCLDEKRELSEKVKHAKRLSDKRNLLQDPNFTSINRQLDRGWRGSTDITIQGGNDVFKENYVTLPGTFDECYPTYLYQKIDESKLKAYTRYELRGYIEDSQDLEVYLIRYNAKHETVNVPGTGSLWPLSVESPIGRCGEPNRCVPHIEWNPDLDCSCRDGEKCAHHSHHFSLDIDVGCTDLNEDLGVWVIFKIKTQDGHARLGNLEFLEEKPLLGEALARVKRAEKKWRDKREQLQFETNIVYKEAKESVDALFVDSHYNRLQADTNITMIHAADKRVHRIREAYLPELSVIPGVNADIFEELEGLIFTAFSLYDARNIIKNGDFNNGLSCWNVKGHVDIQQNDHRSVLVVPEWESEVSQEVRVCPGRGYILRVTAYKEGYGEGCVTIHEIEDNTDELKFSNCIEEEVYPTDTGNDYTAHQGTTGCADACNSRNVGYEDGYEINTTASVNYKPTYEEEMYTDVRRDNHCEYDRGYGNHTPLPAGYVTKELEYFPETDTVWIEIGETEGTFIVDSVELLLMEE

SEQ ID NO: 17 - protein, 1168 aa, Artificial Sequence
  Modified Bt toxin
MEINNQKQCIPYNCLSNPEEVLLDGERILPDIDPLEVSLSLLQFLLNNFVPGGGFISGLVDKIWGALRPSEWDLFLAQIERLIDQRIEATVRAKAIAELEGLGRSYQLYGEAFKEWEKTPDNTAARSRVTERFRIIDAQIEANIPSFRVSGFEVPLLLVYTQAANLHLALLRDSVVFGERWGLTTTNVNDIYNRQVNRIGEYSNHCVDTYNTELERLGFRSIAQWRIYNQFRRELTLTVLDIVALFPNYDSRLYPIQTFSQLTREIVTSPVSEFYYGVINSGNINGTLTEQQIRRPHLMDFFNSMIMYTSDNRREHYWSGLEMTAYFTGFAGAQVSFPLVGTRGESAPPLTVRSVNDGIYRILSAPFYSAPFLGTIVLGSRGEKFDFALNNISPPPSTIYRHPGTVDSLVSIPPQDNSVPPHRGSSHRLSHVTMRASSPIFHWTHRSATPTNTIDPERITQIPLVKAHTLQSGTTVVRGPGFTGGDILRRTSGGPFAYTIVNINGQLPQRYRARIRYASTTNLRIYVTVAGERIFAGQFNKTMDTGDPLTFQSFSYATINTAFTFPMSQSSFTVGADTFSSGNEVYIDRFELIPVTATFEAEYDLERAQKAVNALFTSTNQLGLKTDVTDYQIDQVSNLVECLSDEFCLDEKRELSEKVKHAKRLSDKRNLLQDPNFTSINRQLDRGWRGSTDITIQGGNDVFKENYVTLPGTFDECYPTYLYQKIDESKLKAYTRYELRGYIEDSQDLEVYLIRYNAKHETVNVPGTGSLWPLSVESPIGRCGEPNRCVPHIEWNPDLDCSCRDGEKCAHHSHHFSLDIDVGCTDLNEDLGVWVIFKIKTQDGHARLGNLEFLEEKPLLGEALARVKRAEKKWRDKREQLQFETNIVYKEAKESVDALFVDSHYNRLQADTNITMIHAADKRVHRIREAYLPELSVIPGVNADIFEELEGLIFTAFSLYDARNIIKNGDFNNGLSCWNVKGHVDIQQNDHRSVLVVPEWESEVSQEVRVCPGRGYILRVTAYKEGYGEGCVTIHEIEDNTDELKFSNCIEEEVYPTDTGNDYTAHQGTTGCADACNSRNVGYEDGYEINTTASVNYKPTYEEEMYTDVRRDNHCEYDRGYGNHTPLPAGYVTKELEYFPETDTVWIEIGETEGTFIVDSVELLLMEE

SEQ ID NO: 18 - protein, 1169 aa, Artificial Sequence
  Modified Bt toxin
MEINNQKQCIPYNCLSNPEEVLLDGERILPDIDPLEVSLSLLQFLLNNFVPGGGFISGLVDKIWGALRPSEWDLFLAQIERLIDQRIEATVRAKAIAELEGLGRSYQLYGEAFKEWEKTPDNTAARSRVTERFRIIDAQIEANIPSFRVSGFEVPLLLVYTQAANLHLALLRDSVVFGERWGLTTTNVNDIYNRQVNRIGEYSNHCVDTYNTELERLGFRSIAQWRIYNQFRRELTLTVLDIVALFPNYDSRLYPIQTFSQLTREIVTSPVSEFYYGVINSGNINGTLTEQQIRRPHLMDFFNSMIMYTSDNRREHYWSGLEMTAYFTGFAGAQVSFPLVGTRGESAPPLTVRSVNDGIYRILSAPFYSAPFLGTIVLGSRGEKFDFALNNISPPPSTIYRHPGTVDSLVSIPPQDNSVPPHRGSSHRLSHVTMRASSPIFHWTHRSATTTNTINPNAIIQIPLVKAHTLQSGTTVVRGPGFTGGDILRRTSGGPFAYTIVNINGQLPQRYRARIRYASTTNLRIYVTVAGERIFAGQFNKTMDTGDPLTFQSFSYATINTAFTFPMSQSSFTVGADTFSSGNEVYIDRFELIPVTATFEAEYDLEKAQKAVNALFTSSNQIGLKTDVTDYHIDKVSNLVECLSDEFCLDEKRELSEKVKHAKRLCDERNLLQDPNFRGINRQPDRGWRGSTDITIQGGDDVFKENYVTLPGTFDECYPTYLYQKIDESKLKAYTRYELRGYIEDSQDLEIYLIRYNAKHETVNVPGTGSLWPLSAQSPIGKCGEPNRCATHLEWNPDLDCSCRDGEKCAHHSHHFSLDIDVGCTDLNEDLGVWVIFKIKTQDGHARLGNLEFLEEKPLVGEALARVKRAEKKWRDKREKLELETNIVYKEAKKSVDALFVNSQYDRLQADTNIAIIHAADKRVHSIREAYLPELSVIPGVNAAIFEELEGRIFTAYSLYDARNVIKNGDFNNGLSCWNVKGHVDVEEQNNHRSVLVVPEWEAEVSQEVRVCPGRGYILRVTAYKEGYGEGCVTIHEIEDNTDELKFSNCVEEEIYPNNTVTCNDYTATQEEYEGTYTSRNRGYDGAYESNSSVPADYASAYEEKAYTDGRRDNTCESNRGYGDYTPLPAGYVTKELEYFPETDKVWIEIGETEGTFIVDSVELLLMEE

SEQ ID NO: 19 - DNA, 3510 bp, Artificial Sequence
  Modified Bt toxin
atggagataaataatcagaagcaatgcataccatataattgcttaagtaatcctgaggaagtacttttggatggggagaggatattacctgatatcgatccactcgaagtttctttgtcgcttttgcaatttcttttgaataactttgttccagggggaggctttatttcaggattagttgataaaatatggggggctttgagaccatctgaatgggacttatttcttgcacagattgaacggttgattgatcaaagaatagaagcaacagtaagagcaaaagcaatcgctgaattagaaggtttagggagaagttatcaactatatggagaggcatttaaagagtgggaaaaaactccagataacacagcggctcggtctagagtaactgagagatttcgtataattgatgctcaaattgaagcaaatatcccttcgtttcgggtttccggatttgaagtgccacttctattggtttatacccaagcagctaatttgcatctcgctctattaagagattctgttgtttttggagagagatggggattgacgactacaaatgtcaatgatatctataatagacaagttaatagaattggtgaatatagcaatcattgcgtagatacgtataacacagaactagaacgtctagggtttagatctatagcgcagtggagaatatataatcagtttagaagagaactaacactaactgtattagatattgtcgctcttttcccgaactatgacagtagactgtatccgatccaaactttttctcaattgacaagagaaattgttacatccccagtaagcgaattttattatggtgttattaatagtggtaatataaatggtactcttactgaacagcagataaggcgaccacatcttatggacttctttaactccatgatcatgtatacatcagataatagacgggaacattattggtcaggacttgaaatgacggcttattttacaggatttgcaggcgctcaagtgtcattccctttagtcgggactagaggggagtcagctccaccattaactgttagaagtgttaatgatggaatttatagaatattatcggcaccgttttattcagcgccttttctaggcaccattgtattgggaagtcgtggagaaaaatttgattttgcgcttaataatatttcacctccgccatctacaatatacagacatcctggaacagtagattcactagtcagtataccgccacaggataatagcgtaccaccgcacaggggatctagtcatcgattaagtcatgttacaatgcgcgcaagttcccctatattccattggacgcatcgcagcgcaaccactacaaatacaattaatccaaatgctattatccaaataccgttagtaaaagcacatacacttcagtcaggtactactgttgtaagagggcccgggtttacgggaggagatattcttcgacgaacaagtggaggaccatttgcttatactattgttaatataaatgggcaattaccccaaaggtatcgtgcaagaatacgctatgcctctactacaaatctaagaatttacgtaacggttgcaggtgaacggatttttgctggtcaatttaacaaaacaatggataccggtgacccattaacattccaatcttttagttacgcaactattaatacagcttttacattcccaatgagccagagtagtttcacagtaggtgctgatacttttagttcagggaatgaagtttatatagacagatttgaattgattccagttactgcaacatttgaggcagaatatgatttagagaaagctcagaaagcggtgaatgcgctgtttacttcttccaatcaaatcgggttaaaaacagatgtgacggactatcatattgataaagtatccaatctagttgagtgtttatcagatgaattttgtctagatgaaaagcgagaattgtccgagaaagtcaaacatgcgaagcgactctgtgatgagcggaatttacttcaagatccaaacttcagaggcatcaatagacaaccagaccgtggttggagaggaagtacggatattaccatccaaggaggagatgacgtattcaaagagaattacgttacgctaccgggtacctttgatgagtgctatccaacgtatttatatcaaaaaatagatgagtcgaaattaaaagcctatacccgctatgaattaagagggtatatcgaggatagtcaagacttagaaatctatttaattcgctacaatgcaaaacatgaaacagtaaatgtgccaggtacgggttccttatggccgctttcagcccaaagtccaatcggaaagtgtggagaaccgaatcgatgtgcgacacaccttgaatggaatcctgacttagattgttcgtgtagggatggagaaaagtgtgcccatcattcgcatcatttctccttagacattgatgtaggatgtacagacctaaatgaggacctaggtgtatgggtgatctttaagattaagacgcaagatggtcatgcgagactaggaaatctagaatttctcgaagagaaaccattagtaggagaagcgctagctcgtgtgaagagagcggagaaaaaatggagagacaaacgcgaaaaattggaattggaaacaaatattgtttataaagaggcaaaaaaatctgtagatgctttatttgtgaactctcaatatgatagattacaagcggatacgaatatcgcgataattcatgcggcagataaacgcgttcatagcattcgagaagcatatcttccagagttgtctgtaattccgggtgtaaatgcagctatttttgaagaattagagggacgtattttcacagcctactctctatatgatgcgagaaatgtcattaaaaatggcgatttcaataatggcttatcatgctggaacgtgaaagggcatgtagatgtagaagaacagaacaaccatcgttcggtccttgttgttccagaatgggaagcagaagtgtcacaagaggttcgtgtctgtccaggtcgtggctatatccttcgtgttacagcgtacaaagagggatatggagagggctgtgtaacgattcatgagatcgaagacaatacagacgaactgaaattcagcaactgtgtagaagaggaaatatatccaaacaacacggtaacgtgtaatgattatactgcgactcaagaagaatatgagggtacgtacacttctcgtaatcgaggatatgacggagcctatgaaagcaattcttctgtaccagctgattatgcatcagcctatgaagaaaaagcgtatacagatggaagaagagacaatacttgtgaatctaacagaggatatggggattacacaccactaccagctggctatgtgacaaaagaattagagtacttcccagaaaccgataaggtatggattgagattggagaaacggaaggaacatttatcgtggacagcgtggaattactccttatggaggaatag

SEQ ID NO: 20 - DNA, 3507 bp, Artificial Sequence
  Modified Bt toxin
atggagataaataatcagaagcaatgcataccatataattgcttaagtaatcctgaggaagtacttttggatggggagaggatattacctgatatcgatccactcgaagtttctttgtcgcttttgcaatttcttttgaataactttgttccagggggaggctttatttcaggattagttgataaaatatggggggctttgagaccatctgaatgggacttatttcttgcacagattgaacggttgattgatcaaagaatagaagcaacagtaagagcaaaagcaatcgctgaattagaaggtttagggagaagttatcaactatatggagaggcatttaaagagtgggaaaaaactccagataacacagcggctcggtctagagtaactgagagatttcgtataattgatgctcaaattgaagcaaatatcccttcgtttcgggtttccggatttgaagtgccacttctattggtttatacccaagcagctaatttgcatctcgctctattaagagattctgttgtttttggagagagatggggattgacgactacaaatgtcaatgatatctataatagacaagttaatagaattggtgaatatagcaatcattgcgtagatacgtataacacagaactagaacgtctagggtttagatctatagcgcagtggagaatatataatcagtttagaagagaactaacactaactgtattagatattgtcgctcttttcccgaactatgacagtagactgtatccgatccaaactttttctcaattgacaagagaaattgttacatccccagtaagcgaattttattatggtgttattaatagtggtaatataaatggtactcttactgaacagcagataaggcgaccacatcttatggacttctttaactccatgatcatgtatacatcagataatagacgggaacattattggtcaggacttgaaatgacggcttattttacaggatttgcaggcgctcaagtgtcattccctttagtcgggactagaggggagtcagctccaccattaactgttagaagtgttaatgatggaatttatagaatattatcggcaccgttttattcagcgccttttctaggcaccattgtattgggaagtcgtggagaaaaatttgattttgcgcttaataatatttcacctccgccatctacaatatacagacatcctggaacagtagattcactagtcagtataccgccacaggataatagcgtaccaccgcacaggggatctagtcatcgattaagtcatgttacaatgcgcgcaagttcccctatattccattggacgcatcgcagcgcaaccactacaaatacaattaatccaaatgctattatccaaataccactagtaaaagcacatacacttcagtcaggtactactgttgtaaaagggcccgggtttacgggaggagatattcttcgacgaacaagtggaggaccatttgcttttagtaatgttaatttagactggaatttatcacaaaggtatcgtgcaagaatacgctatgcctctactacaaatctaagaatgtacgtaacgattgcaggtgaacggatttttgctggtcaatttaacaaaacaatgaataccggtgacccattaacattccaatcttttagttacgcaactattgatacagcttttacattcccaacgaaagctagtagtttgacagtaggtgctgatacttttagttcagggaatgaagtttatgtagacagatttgaattgattccagttactgcaacattcgaggcagaatctgatttagaaagagcgcaaaaggcggtgaatgccctgtttacttctacaaaccaactagggctaaaaacagatgtgacggattatcagattgatcaagtgtccaatttagtagaatgtttatcagatgaattttgtctggatgaaaagagagaattgtccgagaaagtcaaacatgcaaagcgacttagtgataagcggaacctacttcaagatccaaacttcacatctatcaatagacaactagaccgtggatggagaggaagtacggatattaccatccaaggaggaaatgacgtattcaaagagaattacgtcacactaccaggtacctttgatgagtgttatccaacgtatttgtatcaaaaaatagatgagtcaaaattaaaagcctatactcgctatgaattaagagggtatattgaagatagtcaagatttagaagtctatttgattcgttacaatgcgaaacatgaaacagtaaatgttcccggtacagggtccttatggccgctttcagtcgaaagcccaatcggaaggtgcggagaaccgaatcgatgtgtgccacatattgaatggaatcctgatttagattgttcgtgtagggatggggagaagtgtgcccatcattcgcatcatttctctctagatattgatgttggatgtacagacctaaatgaggacctaggtgtatgggtgatctttaagattaaaacgcaggatggccatgcaagattaggaaatctagagtttctcgaagagaaaccattgttaggagaagcgttagctcgtgtgaaaagagcggagaaaaaatggagagacaaacgcgaacaattgcagtttgaaacgaatatcgtttacaaagaggcaaaagaatctgtagatgctttattcgtagattctcactataatagattacaagcggatacgaacattacgatgattcatgcggcagataaacgcgttcatcgaatccgagaggcttatcttccggaattatccgttatcccaggtgtaaatgcggacatttttgaagaattagaaggtcttattttcactgcattctccctatatgatgcgagaaatatcattaaaaacggtgatttcaataatggtttatcgtgttggaacgtgaaagggcatgtagatatacaacagaatgatcatcgttctgtcctcgttgtcccggaatgggaatcagaggtatcacaagaagtccgcgtatgtccaggtcgtggctatattcttcgtgtcacagcgtacaaagagggctacggagaaggatgcgtaacgatccatgagatcgaagacaatacagacgaattgaagtttagtaactgcatagaagaggaagtctatccaacggatacaggtaatgattatactgcacaccaaggtacaacaggatgcgcagatgcatgtaattcccgtaatgttggatatgaggatggatatgaaataaatactacagcatctgttaattacaaaccgacttatgaagaagaaatgtatacagatgtacgaagagataatcattgtgaatatgacagaggatatgggaaccatacaccgttaccagctggttatgtaacaaaagaattagagtacttccctgaaacagatacagtatggatagagattggagaaacggaaggaacattcatcgtagatagtgtggaattactcctcatggaggaataa

SEQ ID NO: 21 - DNA, 3507 bp, Artificial Sequence
  Modified Bt toxin
atggagataaataatcagaagcaatgcataccatataattgcttaagtaatcctgaggaagtacttttggatggggagaggatattacctgatatcgatccactcgaagtttctttgtcgcttttgcaatttcttttgaataactttgttccagggggaggctttatttcaggattagttgataaaatatggggggctttgagaccatctgaatgggacttatttcttgcacagattgaacggttgattgatcaaagaatagaagcaacagtaagagcaaaagcaatcgctgaattagaaggtttagggagaagttatcaactatatggagaggcatttaaagagtgggaaaaaactccagataacacagcggctcggtctagagtaactgagagatttcgtataattgatgctcaaattgaagcaaatatcccttcgtttcgggtttccggatttgaagtgccacttctattggtttatacccaagcagctaatttgcatctcgctctattaagagattctgttgtttttggagagagatggggattgacgactacaaatgtcaatgatatctataatagacaagttaatagaattggtgaatatagcaatcattgcgtagatacgtataacacagaactagaacgtctagggtttagatctatagcgcagtggagaatatataatcagtttagaagagaactaacactaactgtattagatattgtcgctcttttcccgaactatgacagtagactgtatccgatccaaactttttctcaattgacaagagaaattgttacatccccagtaagcgaattttattatggtgttattaatagtggtaatataaatggtactcttactgaacagcagataaggcgaccacatcttatggacttctttaactccatgatcatgtatacatcagataatagacgggaacattattggtcaggacttgaaatgacggcttattttacaggatttgcaggcgctcaagtgtcattccctttagtcgggactagaggggagtcagctccaccattaactgttagaagtgttaatgatggaatttatagaatattatcggcaccgttttattcagcgccttttctaggcaccattgtattgggaagtcgtggagaaaaatttgattttgcgcttaataatatttcacctccgccatctacaatatacagacatcctggaacagtagattcactagtcagtataccgccacaggataatagcgtaccaccgcacaggggatctagtcatcgattaagtcatgttacaatgcgcgcaagttcccctatattccattggacgcatcgcagcgcaaccactacaaatacaattcattcagatagtattactcaaataccattggtaaaagcacatacacttcagtcaggtactactgttgtaaaagggcccgggtttacgggaggagatattcttcgacgaacaagtggaggaccatttgcttttagtaatgttaatttagactggaatttatcacaaaggtatcgtgcaagaatacgctatgcctctactacaaatctaagaatgtacgtaacgattgcaggtgaacggatttttgctggtcaatttaacaaaacaatgaataccggtgacccattaacattccaatcttttagttacgcaactattgatacagcttttacattcccaacgaaagctagtagtttgacagtaggtgctgatacttttagttcagggaatgaagtttatgtagacagatttgaattgattccagttactgcaacattcgaggcagaatctgatttagaaagagcgcaaaaggcggtgaatgccctgtttacttctacaaaccaactagggctaaaaacagatgtgacggattatcagattgatcaagtgtccaatttagtagaatgtttatcagatgaattttgtctggatgaaaagagagaattgtccgagaaagtcaaacatgcaaagcgacttagtgataagcggaacctacttcaagatccaaacttcacatctatcaatagacaactagaccgtggatggagaggaagtacggatattaccatccaaggaggaaatgacgtattcaaagagaattacgtcacactaccaggtacctttgatgagtgttatccaacgtatttgtatcaaaaaatagatgagtcaaaattaaaagcctatactcgctatgaattaagagggtatattgaagatagtcaagatttagaagtctatttgattcgttacaatgcgaaacatgaaacagtaaatgttcccggtacagggtccttatggccgctttcagtcgaaagcccaatcggaaggtgcggagaaccgaatcgatgtgtgccacatattgaatggaatcctgatttagattgttcgtgtagggatggggagaagtgtgcccatcattcgcatcatttctctctagatattgatgttggatgtacagacctaaatgaggacctaggtgtatgggtgatctttaagattaaaacgcaggatggccatgcaagattaggaaatctagagtttctcgaagagaaaccattgttaggagaagcgttagctcgtgtgaaaagagcggagaaaaaatggagagacaaacgcgaacaattgcagtttgaaacgaatatcgtttacaaagaggcaaaagaatctgtagatgctttattcgtagattctcactataatagattacaagcggatacgaacattacgatgattcatgcggcagataaacgcgttcatcgaatccgagaggcttatcttccggaattatccgttatcccaggtgtaaatgcggacatttttgaagaattagaaggtcttattttcactgcattctccctatatgatgcgagaaatatcattaaaaacggtgatttcaataatggtttatcgtgttggaacgtgaaagggcatgtagatatacaacagaatgatcatcgttctgtcctcgttgtcccggaatgggaatcagaggtatcacaagaagtccgcgtatgtccaggtcgtggctatattcttcgtgtcacagcgtacaaagagggctacggagaaggatgcgtaacgatccatgagatcgaagacaatacagacgaattgaagtttagtaactgcatagaagaggaagtctatccaacggatacaggtaatgattatactgcacaccaaggtacaacaggatgcgcagatgcatgtaattcccgtaatgttggatatgaggatggatatgaaataaatactacagcatctgttaattacaaaccgacttatgaagaagaaatgtatacagatgtacgaagagataatcattgtgaatatgacagaggatatgggaaccatacaccgttaccagctggttatgtaacaaaagaattagagtacttccctgaaacagatacagtatggatagagattggagaaacggaaggaacattcatcgtagatagtgtggaattactcctcatggaggaataa

SEQ ID NO: 22 - DNA, 3507 bp, Artificial Sequence
  Modified Bt toxin
atggagataaataatcagaagcaatgcataccatataattgcttaagtaatcctgaggaagtacttttggatggggagaggatattacctgatatcgatccactcgaagtttctttgtcgcttttgcaatttcttttgaataactttgttccagggggaggctttatttcaggattagttgataaaatatggggggctttgagaccatctgaatgggacttatttcttgcacagattgaacggttgattgatcaaagaatagaagcaacagtaagagcaaaagcaatcgctgaattagaaggtttagggagaagttatcaactatatggagaggcatttaaagagtgggaaaaaactccagataacacagcggctcggtctagagtaactgagagatttcgtataattgatgctcaaattgaagcaaatatcccttcgtttcgggtttccggatttgaagtgccacttctattggtttatacccaagcagctaatttgcatctcgctctattaagagattctgttgtttttggagagagatggggattgacgactacaaatgtcaatgatatctataatagacaagttaatagaattggtgaatatagcaatcattgcgtagatacgtataacacagaactagaacgtctagggtttagatctatagcgcagtggagaatatataatcagtttagaagagaactaacactaactgtattagatattgtcgctcttttcccgaactatgacagtagactgtatccgatccaaactttttctcaattgacaagagaaattgttacatccccagtaagcgaattttattatggtgttattaatagtggtaatataaatggtactcttactgaacagcagataaggcgaccacatcttatggacttctttaactccatgatcatgtatacatcagataatagacgggaacattattggtcaggacttgaaatgacggcttattttacaggatttgcaggcgctcaagtgtcattccctttagtcgggactagaggggagtcagctccaccattaactgttagaagtgttaatgatggaatttatagaatattatcggcaccgttttattcagcgccttttctaggcaccattgtattgggaagtcgtggagaaaaatttgattttgcgcttaataatatttcacctccgccatctacaatatacagacatcctggaacagtagattcactagtcagtataccgccacaggataatagcgtaccaccgcacaggggatctagtcatcgattaagtcatgttacaatgcgcgcaagttcccctatattccattggacgcatcgcagcgcagatcgtacaaatacaattcattcagatagtattactcaaataccattggtaaaagcacatacacttcagtcaggtactactgttgtaaaagggcccgggtttacgggaggagatattcttcgacgaacaagtggaggaccatttgcttttagtaatgttaatttagactggaatttatcacaaaggtatcgtgcaagaatacgctatgcctctactacaaatctaagaatgtacgtaacgattgcaggtgaacggatttttgctggtcaatttaacaaaacaatgaataccggtgacccattaacattccaatcttttagttacgcaactattgatacagcttttacattcccaacgaaagctagtagtttgacagtaggtgctgatacttttagttcagggaatgaagtttatgtagacagatttgaattgattccagttactgcaacattcgaggcagaatctgatttagaaagagcgcaaaaggcggtgaatgccctgtttacttctacaaaccaactagggctaaaaacagatgtgacggattatcagattgatcaagtgtccaatttagtagaatgtttatcagatgaattttgtctggatgaaaagagagaattgtccgagaaagtcaaacatgcaaagcgacttagtgataagcggaacctacttcaagatccaaacttcacatctatcaatagacaactagaccgtggatggagaggaagtacggatattaccatccaaggaggaaatgacgtattcaaagagaattacgtcacactaccaggtacctttgatgagtgttatccaacgtatttgtatcaaaaaatagatgagtcaaaattaaaagcctatactcgctatgaattaagagggtatattgaagatagtcaagatttagaagtctatttgattcgttacaatgcgaaacatgaaacagtaaatgttcccggtacagggtccttatggccgctttcagtcgaaagcccaatcggaaggtgcggagaaccgaatcgatgtgtgccacatattgaatggaatcctgatttagattgttcgtgtagggatggggagaagtgtgcccatcattcgcatcatttctctctagatattgatgttggatgtacagacctaaatgaggacctaggtgtatgggtgatctttaagattaaaacgcaggatggccatgcaagattaggaaatctagagtttctcgaagagaaaccattgttaggagaagcgttagctcgtgtgaaaagagcggagaaaaaatggagagacaaacgcgaacaattgcagtttgaaacgaatatcgtttacaaagaggcaaaagaatctgtagatgctttattcgtagattctcactataatagattacaagcggatacgaacattacgatgattcatgcggcagataaacgcgttcatcgaatccgagaggcttatcttccggaattatccgttatcccaggtgtaaatgcggacatttttgaagaattagaaggtcttattttcactgcattctccctatatgatgcgagaaatatcattaaaaacggtgatttcaataatggtttatcgtgttggaacgtgaaagggcatgtagatatacaacagaatgatcatcgttctgtcctcgttgtcccggaatgggaatcagaggtatcacaagaagtccgcgtatgtccaggtcgtggctatattcttcgtgtcacagcgtacaaagagggctacggagaaggatgcgtaacgatccatgagatcgaagacaatacagacgaattgaagtttagtaactgcatagaagaggaagtctatccaacggatacaggtaatgattatactgcacaccaaggtacaacaggatgcgcagatgcatgtaattcccgtaatgttggatatgaggatggatatgaaataaatactacagcatctgttaattacaaaccgacttatgaagaagaaatgtatacagatgtacgaagagataatcattgtgaatatgacagaggatatgggaaccatacaccgttaccagctggttatgtaacaaaagaattagagtacttccctgaaacagatacagtatggatagagattggagaaacggaaggaacattcatcgtagatagtgtggaattactcctcatggaggaataa

SEQ ID NO: 23 - DNA, 3507 bp, Artificial Sequence
  Modified Bt toxin
atggagataaataatcagaagcaatgcataccatataattgcttaagtaatcctgaggaagtacttttggatggggagaggatattacctgatatcgatccactcgaagtttctttgtcgcttttgcaatttcttttgaataactttgttccagggggaggctttatttcaggattagttgataaaatatggggggctttgagaccatctgaatgggacttatttcttgcacagattgaacggttgattgatcaaagaatagaagcaacagtaagagcaaaagcaatcgctgaattagaaggtttagggagaagttatcaactatatggagaggcatttaaagagtgggaaaaaactccagataacacagcggctcggtctagagtaactgagagatttcgtataattgatgctcaaattgaagcaaatatcccttcgtttcgggtttccggatttgaagtgccacttctattggtttatacccaagcagctaatttgcatctcgctctattaagagattctgttgtttttggagagagatggggattgacgactacaaatgtcaatgatatctataatagacaagttaatagaattggtgaatatagcaatcattgcgtagatacgtataacacagaactagaacgtctagggtttagatctatagcgcagtggagaatatataatcagtttagaagagaactaacactaactgtattagatattgtcgctcttttcccgaactatgacagtagactgtatccgatccaaactttttctcaattgacaagagaaattgttacatccccagtaagcgaattttattatggtgttattaatagtggtaatataaatggtactcttactgaacagcagataaggcgaccacatcttatggacttctttaactccatgatcatgtatacatcagataatagacgggaacattattggtcaggacttgaaatgacggcttattttacaggatttgcaggcgctcaagtgtcattccctttagtcgggactagaggggagtcagctccaccattaactgttagaagtgttaatgatggaatttatagaatattatcggcaccgttttattcagcgccttttctaggcaccattgtattgggaagtcgtggagaaaaatttgattttgcgcttaataatatttcacctccgccatctacaatatacagacatcctggaacagtagattcactagtcagtataccgccacaggataatagcgtaccaccgcacaggggatctagtcatcgattaagtcatgttacaatgcgcgcaagttcccctatattccattggacgcatcgcagcgcaaccactacaaatacaattaatccaaatgctattatccaaataccactagtaaaagcacatacacttcagtcaggtactactgttgtaaaagggcccgggtttacgggaggagatattcttcgacgaacaagtggaggaccatttgcttttagtaatgttaatttagactggaatttatcacaaaggtatcgtgcaagaatacgctatgcctctactacaaatctaagaatgtacgtaacgattgcaggtgaacggatttttgctggtcaatttaacaaaacaatgaataccggtgacccattaacattccaatcttttagttacgcaactattgatacagcttttacattcccaacgaaagctagtagtttgacagtaggtgctgatacttttagttcagggaatgaagtttatgtagacagatttgaattgattccagttactgcaacacttgaagcagtaactgatttagaaagagcgcaaaaggcggtgaatgccctgtttacttctacaaaccaactagggctaaaaacagatgtgacggattatcagattgatcaagtgtccaatttagtagaatgtttatcagatgaattttgtctggatgaaaagagagaattgtccgagaaagtcaaacatgcaaagcgacttagtgataagcggaacctacttcaagatccaaacttcacatctatcaatagacaactagaccgtggatggagaggaagtacggatattaccatccaaggaggaaatgacgtattcaaagagaattacgtcacactaccaggtacctttgatgagtgttatccaacgtatttgtatcaaaaaatagatgagtcaaaattaaaagcctatactcgctatgaattaagagggtatattgaagatagtcaagatttagaagtctatttgattcgttacaatgcgaaacatgaaacagtaaatgttcccggtacagggtccttatggccgctttcagtcgaaagcccaatcggaaggtgcggagaaccgaatcgatgtgtgccacatattgaatggaatcctgatttagattgttcgtgtagggatggggagaagtgtgcccatcattcgcatcatttctctctagatattgatgttggatgtacagacctaaatgaggacctaggtgtatgggtgatctttaagattaaaacgcaggatggccatgcaagattaggaaatctagagtttctcgaagagaaaccattgttaggagaagcgttagctcgtgtgaaaagagcggagaaaaaatggagagacaaacgcgaacaattgcagtttgaaacgaatatcgtttacaaagaggcaaaagaatctgtagatgctttattcgtagattctcactataatagattacaagcggatacgaacattacgatgattcatgcggcagataaacgcgttcatcgaatccgagaggcttatcttccggaattatccgttatcccaggtgtaaatgcggacatttttgaagaattagaaggtcttattttcactgcattctccctatatgatgcgagaaatatcattaaaaacggtgatttcaataatggtttatcgtgttggaacgtgaaagggcatgtagatatacaacagaatgatcatcgttctgtcctcgttgtcccggaatgggaatcagaggtatcacaagaagtccgcgtatgtccaggtcgtggctatattcttcgtgtcacagcgtacaaagagggctacggagaaggatgcgtaacgatccatgagatcgaagacaatacagacgaattgaagtttagtaactgcatagaagaggaagtctatccaacggatacaggtaatgattatactgcacaccaaggtacaacaggatgcgcagatgcatgtaattcccgtaatgttggatatgaggatggatatgaaataaatactacagcatctgttaattacaaaccgacttatgaagaagaaatgtatacagatgtacgaagagataatcattgtgaatatgacagaggatatgggaaccatacaccgttaccagctggttatgtaacaaaagaattagagtacttccctgaaacagatacagtatggatagagattggagaaacggaaggaacattcatcgtagatagtgtggaattactcctcatggaggaataa

SEQ ID NO: 24 - DNA, 3507 bp, Artificial Sequence
  Modified Bt toxin
atggagataaataatcagaagcaatgcataccatataattgcttaagtaatcctgaggaagtacttttggatggggagaggatattacctgatatcgatccactcgaagtttctttgtcgcttttgcaatttcttttgaataactttgttccagggggaggctttatttcaggattagttgataaaatatggggggctttgagaccatctgaatgggacttatttcttgcacagattgaacggttgattgatcaaagaatagaagcaacagtaagagcaaaagcaatcgctgaattagaaggtttagggagaagttatcaactatatggagaggcatttaaagagtgggaaaaaactccagataacacagcggctcggtctagagtaactgagagatttcgtataattgatgctcaaattgaagcaaatatcccttcgtttcgggtttccggatttgaagtgccacttctattggtttatacccaagcagctaatttgcatctcgctctattaagagattctgttgtttttggagagagatggggattgacgactacaaatgtcaatgatatctataatagacaagttaatagaattggtgaatatagcaatcattgcgtagatacgtataacacagaactagaacgtctagggtttagatctatagcgcagtggagaatatataatcagtttagaagagaactaacactaactgtattagatattgtcgctcttttcccgaactatgacagtagactgtatccgatccaaactttttctcaattgacaagagaaattgttacatccccagtaagcgaattttattatggtgttattaatagtggtaatataaatggtactcttactgaacagcagataaggcgaccacatcttatggacttctttaactccatgatcatgtatacatcagataatagacgggaacattattggtcaggacttgaaatgacggcttattttacaggatttgcaggcgctcaagtgtcattccctttagtcgggactagaggggagtcagctccaccattaactgttagaagtgttaatgatggaatttatagaatattatcggcaccgttttattcagcgccttttctaggcaccattgtattgggaagtcgtggagaaaaatttgattttgcgcttaataatatttcacctccgccatctacaatatacagacatcctggaacagtagattcactagtcagtataccgccacaggataatagcgtaccaccgcacaggggatctagtcatcgattaagtcatgttacaatgcgcgcaagttcccctatattccattggacgcatcgcagcgcaaccactacaaatacaattcattcagatagtattactcaaataccattggtaaaagcacatacacttcagtcaggtactactgttgtaaaagggcccgggtttacgggaggagatattcttcgacgaacaagtggaggaccatttgcttttagtaatgttaatttagactggaatttatcacaaaggtatcgtgcaagaatacgctatgcctctactacaaatctaagaatgtacgtaacgattgcaggtgaacggatttttgctggtcaatttaacaaaacaatgaataccggtgacccattaacattccaatcttttagttacgcaactattgatacagcttttacattcccaacgaaagctagtagtttgacagtaggtgctgatacttttagttcagggaatgaagtttatgtagacagatttgaattgattccagttactgcaacacttgaagcagtaactgatttagaaagagcgcaaaaggcggtgaatgccctgtttacttctacaaaccaactagggctaaaaacagatgtgacggattatcagattgatcaagtgtccaatttagtagaatgtttatcagatgaattttgtctggatgaaaagagagaattgtccgagaaagtcaaacatgcaaagcgacttagtgataagcggaacctacttcaagatccaaacttcacatctatcaatagacaactagaccgtggatggagaggaagtacggatattaccatccaaggaggaaatgacgtattcaaagagaattacgtcacactaccaggtacctttgatgagtgttatccaacgtatttgtatcaaaaaatagatgagtcaaaattaaaagcctatactcgctatgaattaagagggtatattgaagatagtcaagatttagaagtctatttgattcgttacaatgcgaaacatgaaacagtaaatgttcccggtacagggtccttatggccgctttcagtcgaaagcccaatcggaaggtgcggagaaccgaatcgatgtgtgccacatattgaatggaatcctgatttagattgttcgtgtagggatggggagaagtgtgcccatcattcgcatcatttctctctagatattgatgttggatgtacagacctaaatgaggacctaggtgtatgggtgatctttaagattaaaacgcaggatggccatgcaagattaggaaatctagagtttctcgaagagaaaccattgttaggagaagcgttagctcgtgtgaaaagagcggagaaaaaatggagagacaaacgcgaacaattgcagtttgaaacgaatatcgtttacaaagaggcaaaagaatctgtagatgctttattcgtagattctcactataatagattacaagcggatacgaacattacgatgattcatgcggcagataaacgcgttcatcgaatccgagaggcttatcttccggaattatccgttatcccaggtgtaaatgcggacatttttgaagaattagaaggtcttattttcactgcattctccctatatgatgcgagaaatatcattaaaaacggtgatttcaataatggtttatcgtgttggaacgtgaaagggcatgtagatatacaacagaatgatcatcgttctgtcctcgttgtcccggaatgggaatcagaggtatcacaagaagtccgcgtatgtccaggtcgtggctatattcttcgtgtcacagcgtacaaagagggctacggagaaggatgcgtaacgatccatgagatcgaagacaatacagacgaattgaagtttagtaactgcatagaagaggaagtctatccaacggatacaggtaatgattatactgcacaccaaggtacaacaggatgcgcagatgcatgtaattcccgtaatgttggatatgaggatggatatgaaataaatactacagcatctgttaattacaaaccgacttatgaagaagaaatgtatacagatgtacgaagagataatcattgtgaatatgacagaggatatgggaaccatacaccgttaccagctggttatgtaacaaaagaattagagtacttccctgaaacagatacagtatggatagagattggagaaacggaaggaacattcatcgtagatagtgtggaattactcctcatggaggaataa

SEQ ID NO: 25 - DNA, 3507 bp, Artificial Sequence
  Modified Bt toxin
atggagataaataatcagaagcaatgcataccatataattgcttaagtaatcctgaggaagtacttttggatggggagaggatattacctgatatcgatccactcgaagtttctttgtcgcttttgcaatttcttttgaataactttgttccagggggaggctttatttcaggattagttgataaaatatggggggctttgagaccatctgaatgggacttatttcttgcacagattgaacggttgattgatcaaagaatagaagcaacagtaagagcaaaagcaatcgctgaattagaaggtttagggagaagttatcaactatatggagaggcatttaaagagtgggaaaaaactccagataacacagcggctcggtctagagtaactgagagatttcgtataattgatgctcaaattgaagcaaatatcccttcgtttcgggtttccggatttgaagtgccacttctattggtttatacccaagcagctaatttgcatctcgctctattaagagattctgttgtttttggagagagatggggattgacgactacaaatgtcaatgatatctataatagacaagttaatagaattggtgaatatagcaatcattgcgtagatacgtataacacagaactagaacgtctagggtttagatctatagcgcagtggagaatatataatcagtttagaagagaactaacactaactgtattagatattgtcgctcttttcccgaactatgacagtagactgtatccgatccaaactttttctcaattgacaagagaaattgttacatccccagtaagcgaattttattatggtgttattaatagtggtaatataaatggtactcttactgaacagcagataaggcgaccacatcttatggacttctttaactccatgatcatgtatacatcagataatagacgggaacattattggtcaggacttgaaatgacggcttattttacaggatttgcaggcgctcaagtgtcattccctttagtcgggactagaggggagtcagctccaccattaactgttagaagtgttaatgatggaatttatagaatattatcggcaccgttttattcagcgccttttctaggcaccattgtattgggaagtcgtggagaaaaatttgattttgcgcttaataatatttcacctccgccatctacaatatacagacatcctggaacagtagattcactagtcagtataccgccacaggataatagcgtaccaccgcacaggggatctagtcatcgattaagtcatgttacaatgcgcgcaagttcccctatattccattggacgcatcgcagcgcagatcgtacaaatacaattcattcagatagtattactcaaataccattggtaaaagcacatacacttcagtcaggtactactgttgtaaaagggcccgggtttacgggaggagatattcttcgacgaacaagtggaggaccatttgcttttagtaatgttaatttagactggaatttatcacaaaggtatcgtgcaagaatacgctatgcctctactacaaatctaagaatgtacgtaacgattgcaggtgaacggatttttgctggtcaatttaacaaaacaatgaataccggtgacccattaacattccaatcttttagttacgcaactattgatacagcttttacattcccaacgaaagctagtagtttgacagtaggtgctgatacttttagttcagggaatgaagtttatgtagacagatttgaattgattccagttactgcaacacttgaagcagtaactgatttagaaagagcgcaaaaggcggtgaatgccctgtttacttctacaaaccaactagggctaaaaacagatgtgacggattatcagattgatcaagtgtccaatttagtagaatgtttatcagatgaattttgtctggatgaaaagagagaattgtccgagaaagtcaaacatgcaaagcgacttagtgataagcggaacctacttcaagatccaaacttcacatctatcaatagacaactagaccgtggatggagaggaagtacggatattaccatccaaggaggaaatgacgtattcaaagagaattacgtcacactaccaggtacctttgatgagtgttatccaacgtatttgtatcaaaaaatagatgagtcaaaattaaaagcctatactcgctatgaattaagagggtatattgaagatagtcaagatttagaagtctatttgattcgttacaatgcgaaacatgaaacagtaaatgttcccggtacagggtccttatggccgctttcagtcgaaagcccaatcggaaggtgcggagaaccgaatcgatgtgtgccacatattgaatggaatcctgatttagattgttcgtgtagggatggggagaagtgtgcccatcattcgcatcatttctctctagatattgatgttggatgtacagacctaaatgaggacctaggtgtatgggtgatctttaagattaaaacgcaggatggccatgcaagattaggaaatctagagtttctcgaagagaaaccattgttaggagaagcgttagctcgtgtgaaaagagcggagaaaaaatggagagacaaacgcgaacaattgcagtttgaaacgaatatcgtttacaaagaggcaaaagaatctgtagatgctttattcgtagattctcactataatagattacaagcggatacgaacattacgatgattcatgcggcagataaacgcgttcatcgaatccgagaggcttatcttccggaattatccgttatcccaggtgtaaatgcggacatttttgaagaattagaaggtcttattttcactgcattctccctatatgatgcgagaaatatcattaaaaacggtgatttcaataatggtttatcgtgttggaacgtgaaagggcatgtagatatacaacagaatgatcatcgttctgtcctcgttgtcccggaatgggaatcagaggtatcacaagaagtccgcgtatgtccaggtcgtggctatattcttcgtgtcacagcgtacaaagagggctacggagaaggatgcgtaacgatccatgagatcgaagacaatacagacgaattgaagtttagtaactgcatagaagaggaagtctatccaacggatacaggtaatgattatactgcacaccaaggtacaacaggatgcgcagatgcatgtaattcccgtaatgttggatatgaggatggatatgaaataaatactacagcatctgttaattacaaaccgacttatgaagaagaaatgtatacagatgtacgaagagataatcattgtgaatatgacagaggatatgggaaccatacaccgttaccagctggttatgtaacaaaagaattagagtacttccctgaaacagatacagtatggatagagattggagaaacggaaggaacattcatcgtagatagtgtggaattactcctcatggaggaataa

SEQ ID NO: 26 - DNA, 3507 bp, Artificial Sequence
  Modified Bt toxin
atggagataaataatcagaagcaatgcataccatataattgcttaagtaatcctgaggaagtacttttggatggggagaggatattacctgatatcgatccactcgaagtttctttgtcgcttttgcaatttcttttgaataactttgttccagggggaggctttatttcaggattagttgataaaatatggggggctttgagaccatctgaatgggacttatttcttgcacagattgaacggttgattgatcaaagaatagaagcaacagtaagagcaaaagcaatcgctgaattagaaggtttagggagaagttatcaactatatggagaggcatttaaagagtgggaaaaaactccagataacacagcggctcggtctagagtaactgagagatttcgtataattgatgctcaaattgaagcaaatatcccttcgtttcgggtttccggatttgaagtgccacttctattggtttatacccaagcagctaatttgcatctcgctctattaagagattctgttgtttttggagagagatggggattgacgactacaaatgtcaatgatatctataatagacaagttaatagaattggtgaatatagcaatcattgcgtagatacgtataacacagaactagaacgtctagggtttagatctatagcgcagtggagaatatataatcagtttagaagagaactaacactaactgtattagatattgtcgctcttttcccgaactatgacagtagactgtatccgatccaaactttttctcaattgacaagagaaattgttacatccccagtaagcgaattttattatggtgttattaatagtggtaatataaatggtactcttactgaacagcagataaggcgaccacatcttatggacttctttaactccatgatcatgtatacatcagataatagacgggaacattattggtcaggacttgaaatgacggcttattttacaggatttgcaggcgctcaagtgtcattccctttagtcgggactagaggggagtcagctccaccattaactgttagaagtgttaatgatggaatttatagaatattatcggcaccgttttattcagcgccttttctaggcaccattgtattgggaagtcgtggagaaaaatttgattttgcgcttaataatatttcacctccgccatctacaatatacagacatcctggaacagtagattcactagtcagtataccgccacaggataatagcgtaccaccgcacaggggatctagtcatcgattaagtcatgttacaatgcgcgcaagttcccctatattccattggacgcatcgcagcgcaaccactacaaatacaattcattcagatagtattactcaaataccattggtaaaagcacatacacttcagtcaggtactactgttgtaaaagggcccgggtttacgggaggagatattcttcgacgaacaagtggaggaccatttgcttttagtaatgttaatttagactggaatttatcacaaaggtatcgtgcaagaatacgctatgcctctactacaaatctaagaatgtacgtaacgattgcaggtgaacggatttttgctggtcaatttaacaaaacaatgaataccggtgacccattaacattccaatcttttagttacgcaactattgatacagcttttacattcccaacgaaagctagtagtttgacagtaggtgctgatacttttagttcagggaatgaagtttatgtagacagatttgaattgattccagttactgcaacattcgaggcagaatatgatttagaaagagcgcaaaaggcggtgaatgccctgtttacttctacaaaccaactagggctaaaaacagatgtgacggattatcagattgatcaagtgtccaatttagtagaatgtttatcagatgaattttgtctggatgaaaagagagaattgtccgagaaagtcaaacatgcaaagcgacttagtgataagcggaacctacttcaagatccaaacttcacatctatcaatagacaactagaccgtggatggagaggaagtacggatattaccatccaaggaggaaatgacgtattcaaagagaattacgtcacactaccaggtacctttgatgagtgttatccaacgtatttgtatcaaaaaatagatgagtcaaaattaaaagcctatactcgctatgaattaagagggtatattgaagatagtcaagatttagaagtctatttgattcgttacaatgcgaaacatgaaacagtaaatgttcccggtacagggtccttatggccgctttcagtcgaaagcccaatcggaaggtgcggagaaccgaatcgatgtgtgccacatattgaatggaatcctgatttagattgttcgtgtagggatggggagaagtgtgcccatcattcgcatcatttctctctagatattgatgttggatgtacagacctaaatgaggacctaggtgtatgggtgatctttaagattaaaacgcaggatggccatgcaagattaggaaatctagagtttctcgaagagaaaccattgttaggagaagcgttagctcgtgtgaaaagagcggagaaaaaatggagagacaaacgcgaacaattgcagtttgaaacgaatatcgtttacaaagaggcaaaagaatctgtagatgctttattcgtagattctcactataatagattacaagcggatacgaacattacgatgattcatgcggcagataaacgcgttcatcgaatccgagaggcttatcttccggaattatccgttatcccaggtgtaaatgcggacatttttgaagaattagaaggtcttattttcactgcattctccctatatgatgcgagaaatatcattaaaaacggtgatttcaataatggtttatcgtgttggaacgtgaaagggcatgtagatatacaacagaatgatcatcgttctgtcctcgttgtcccggaatgggaatcagaggtatcacaagaagtccgcgtatgtccaggtcgtggctatattcttcgtgtcacagcgtacaaagagggctacggagaaggatgcgtaacgatccatgagatcgaagacaatacagacgaattgaagtttagtaactgcatagaagaggaagtctatccaacggatacaggtaatgattatactgcacaccaaggtacaacaggatgcgcagatgcatgtaattcccgtaatgttggatatgaggatggatatgaaataaatactacagcatctgttaattacaaaccgacttatgaagaagaaatgtatacagatgtacgaagagataatcattgtgaatatgacagaggatatgggaaccatacaccgttaccagctggttatgtaacaaaagaattagagtacttccctgaaacagatacagtatggatagagattggagaaacggaaggaacattcatcgtagatagtgtggaattactcctcatggaggaataa

SEQ ID NO: 27 - DNA, 3507 bp, Artificial Sequence
  Modified Bt toxin
atggagataaataatcagaagcaatgcataccatataattgcttaagtaatcctgaggaagtacttttggatggggagaggatattacctgatatcgatccactcgaagtttctttgtcgcttttgcaatttcttttgaataactttgttccagggggaggctttatttcaggattagttgataaaatatggggggctttgagaccatctgaatgggacttatttcttgcacagattgaacggttgattgatcaaagaatagaagcaacagtaagagcaaaagcaatcgctgaattagaaggtttagggagaagttatcaactatatggagaggcatttaaagagtgggaaaaaactccagataacacagcggctcggtctagagtaactgagagatttcgtataattgatgctcaaattgaagcaaatatcccttcgtttcgggtttccggatttgaagtgccacttctattggtttatacccaagcagctaatttgcatctcgctctattaagagattctgttgtttttggagagagatggggattgacgactacaaatgtcaatgatatctataatagacaagttaatagaattggtgaatatagcaatcattgcgtagatacgtataacacagaactagaacgtctagggtttagatctatagcgcagtggagaatatataatcagtttagaagagaactaacactaactgtattagatattgtcgctcttttcccgaactatgacagtagactgtatccgatccaaactttttctcaattgacaagagaaattgttacatccccagtaagcgaattttattatggtgttattaatagtggtaatataaatggtactcttactgaacagcagataaggcgaccacatcttatggacttctttaactccatgatcatgtatacatcagataatagacgggaacattattggtcaggacttgaaatgacggcttattttacaggatttgcaggcgctcaagtgtcattccctttagtcgggactagaggggagtcagctccaccattaactgttagaagtgttaatgatggaatttatagaatattatcggcaccgttttattcagcgccttttctaggcaccattgtattgggaagtcgtggagaaaaatttgattttgcgcttaataatatttcacctccgccatctacaatatacagacatcctggaacagtagattcactagtcagtataccgccacaggataatagcgtaccaccgcacaggggatctagtcatcgattaagtcatgttacaatgcgcgcaagttcccctatattccattggacgcatcgcagcgcagatcgtacaaatacaattcattcagatagtattactcaaataccattggtaaaagcacatacacttcagtcaggtactactgttgtaaaagggcccgggtttacgggaggagatattcttcgacgaacaagtggaggaccatttgcttttagtaatgttaatttagactggaatttatcacaaaggtatcgtgcaagaatacgctatgcctctactacaaatctaagaatgtacgtaacgattgcaggtgaacggatttttgctggtcaatttaacaaaacaatgaataccggtgacccattaacattccaatcttttagttacgcaactattgatacagcttttacattcccaacgaaagctagtagtttgacagtaggtgctgatacttttagttcagggaatgaagtttatgtagacagatttgaattgattccagttactgcaacattcgaggcagaatatgatttagaaagagcgcaaaaggcggtgaatgccctgtttacttctacaaaccaactagggctaaaaacagatgtgacggattatcagattgatcaagtgtccaatttagtagaatgtttatcagatgaattttgtctggatgaaaagagagaattgtccgagaaagtcaaacatgcaaagcgacttagtgataagcggaacctacttcaagatccaaacttcacatctatcaatagacaactagaccgtggatggagaggaagtacggatattaccatccaaggaggaaatgacgtattcaaagagaattacgtcacactaccaggtacctttgatgagtgttatccaacgtatttgtatcaaaaaatagatgagtcaaaattaaaagcctatactcgctatgaattaagagggtatattgaagatagtcaagatttagaagtctatttgattcgttacaatgcgaaacatgaaacagtaaatgttcccggtacagggtccttatggccgctttcagtcgaaagcccaatcggaaggtgcggagaaccgaatcgatgtgtgccacatattgaatggaatcctgatttagattgttcgtgtagggatggggagaagtgtgcccatcattcgcatcatttctctctagatattgatgttggatgtacagacctaaatgaggacctaggtgtatgggtgatctttaagattaaaacgcaggatggccatgcaagattaggaaatctagagtttctcgaagagaaaccattgttaggagaagcgttagctcgtgtgaaaagagcggagaaaaaatggagagacaaacgcgaacaattgcagtttgaaacgaatatcgtttacaaagaggcaaaagaatctgtagatgctttattcgtagattctcactataatagattacaagcggatacgaacattacgatgattcatgcggcagataaacgcgttcatcgaatccgagaggcttatcttccggaattatccgttatcccaggtgtaaatgcggacatttttgaagaattagaaggtcttattttcactgcattctccctatatgatgcgagaaatatcattaaaaacggtgatttcaataatggtttatcgtgttggaacgtgaaagggcatgtagatatacaacagaatgatcatcgttctgtcctcgttgtcccggaatgggaatcagaggtatcacaagaagtccgcgtatgtccaggtcgtggctatattcttcgtgtcacagcgtacaaagagggctacggagaaggatgcgtaacgatccatgagatcgaagacaatacagacgaattgaagtttagtaactgcatagaagaggaagtctatccaacggatacaggtaatgattatactgcacaccaaggtacaacaggatgcgcagatgcatgtaattcccgtaatgttggatatgaggatggatatgaaataaatactacagcatctgttaattacaaaccgacttatgaagaagaaatgtatacagatgtacgaagagataatcattgtgaatatgacagaggatatgggaaccatacaccgttaccagctggttatgtaacaaaagaattagagtacttccctgaaacagatacagtatggatagagattggagaaacggaaggaacattcatcgtagatagtgtggaattactcctcatggaggaataa

SEQ ID NO: 28 - DNA, 3507 bp, Artificial Sequence
  Modified Bt toxin
atggagataaataatcagaagcaatgcataccatataattgcttaagtaatcctgaggaagtacttttggatggggagaggatattacctgatatcgatccactcgaagtttctttgtcgcttttgcaatttcttttgaataactttgttccagggggaggctttatttcaggattagttgataaaatatggggggctttgagaccatctgaatgggacttatttcttgcacagattgaacggttgattgatcaaagaatagaagcaacagtaagagcaaaagcaatcgctgaattagaaggtttagggagaagttatcaactatatggagaggcatttaaagagtgggaaaaaactccagataacacagcggctcggtctagagtaactgagagatttcgtataattgatgctcaaattgaagcaaatatcccttcgtttcgggtttccggatttgaagtgccacttctattggtttatacccaagcagctaatttgcatctcgctctattaagagattctgttgtttttggagagagatggggattgacgactacaaatgtcaatgatatctataatagacaagttaatagaattggtgaatatagcaatcattgcgtagatacgtataacacagaactagaacgtctagggtttagatctatagcgcagtggagaatatataatcagtttagaagagaactaacactaactgtattagatattgtcgctcttttcccgaactatgacagtagactgtatccgatccaaactttttctcaattgacaagagaaattgttacatccccagtaagcgaattttattatggtgttattaatagtggtaatataaatggtactcttactgaacagcagataaggcgaccacatcttatggacttctttaactccatgatcatgtatacatcagataatagacgggaacattattggtcaggacttgaaatgacggcttattttacaggatttgcaggcgctcaagtgtcattccctttagtcgggactagaggggagtcagctccaccattaactgttagaagtgttaatgatggaatttatagaatattatcggcaccgttttattcagcgccttttctaggcaccattgtattgggaagtcgtggagaaaaatttgattttgcgcttaataatatttcacctccgccatctacaatatacagacatcctggaacagtagattcactagtcagtataccgccacaggataatagcgtaccaccgcacaggggatctagtcatcgattaagtcatgttacaatgcgcgcaagttcccctatattccattggacgcatcgcagcgcaaccactacaaatacaattaatccaaatgctattatccaaataccactagtaaaagcacatacacttcagtcaggtactactgttgtaagagggcccgggtttacgggaggagatattcttcgacgaacaagtggaggaccatttgcttatactattgttaatataaatgggcaattaccccaaaggtatcgtgcaagaatacgctatgcctctactacaaatctaagaatttacgtaacggttgcaggtgaacggatttttgctggtcaatttaacaaaacaatggataccggtgacccattaacattccaatcttttagttacgcaactattaatacagcttttacattcccaatgagccagagtagtttcacagtaggtgctgatacttttagttcagggaatgaagtttatatagacagatttgaattgattccagttactgcaacattcgaggcagaatctgatttagaaagagcgcaaaaggcggtgaatgccctgtttacttctacaaaccaactagggctaaaaacagatgtgacggattatcagattgatcaagtgtccaatttagtagaatgtttatcagatgaattttgtctggatgaaaagagagaattgtccgagaaagtcaaacatgcaaagcgacttagtgataagcggaacctacttcaagatccaaacttcacatctatcaatagacaactagaccgtggatggagaggaagtacggatattaccatccaaggaggaaatgacgtattcaaagagaattacgtcacactaccaggtacctttgatgagtgttatccaacgtatttgtatcaaaaaatagatgagtcaaaattaaaagcctatactcgctatgaattaagagggtatattgaagatagtcaagatttagaagtctatttgattcgttacaatgcgaaacatgaaacagtaaatgttcccggtacagggtccttatggccgctttcagtcgaaagcccaatcggaaggtgcggagaaccgaatcgatgtgtgccacatattgaatggaatcctgatttagattgttcgtgtagggatggggagaagtgtgcccatcattcgcatcatttctctctagatattgatgttggatgtacagacctaaatgaggacctaggtgtatgggtgatctttaagattaaaacgcaggatggccatgcaagattaggaaatctagagtttctcgaagagaaaccattgttaggagaagcgttagctcgtgtgaaaagagcggagaaaaaatggagagacaaacgcgaacaattgcagtttgaaacgaatatcgtttacaaagaggcaaaagaatctgtagatgctttattcgtagattctcactataatagattacaagcggatacgaacattacgatgattcatgcggcagataaacgcgttcatcgaatccgagaggcttatcttccggaattatccgttatcccaggtgtaaatgcggacatttttgaagaattagaaggtcttattttcactgcattctccctatatgatgcgagaaatatcattaaaaacggtgatttcaataatggtttatcgtgttggaacgtgaaagggcatgtagatatacaacagaatgatcatcgttctgtcctcgttgtcccggaatgggaatcagaggtatcacaagaagtccgcgtatgtccaggtcgtggctatattcttcgtgtcacagcgtacaaagagggctacggagaaggatgcgtaacgatccatgagatcgaagacaatacagacgaattgaagtttagtaactgcatagaagaggaagtctatccaacggatacaggtaatgattatactgcacaccaaggtacaacaggatgcgcagatgcatgtaattcccgtaatgttggatatgaggatggatatgaaataaatactacagcatctgttaattacaaaccgacttatgaagaagaaatgtatacagatgtacgaagagataatcattgtgaatatgacagaggatatgggaaccatacaccgttaccagctggttatgtaacaaaagaattagagtacttccctgaaacagatacagtatggatagagattggagaaacggaaggaacattcatcgtagatagtgtggaattactcctcatggaggaataa

SEQ ID NO: 29 - DNA, 3507 bp, Artificial Sequence
  Modified Bt toxin
atggagataaataatcagaagcaatgcataccatataattgcttaagtaatcctgaggaagtacttttggatggggagaggatattacctgatatcgatccactcgaagtttctttgtcgcttttgcaatttcttttgaataactttgttccagggggaggctttatttcaggattagttgataaaatatggggggctttgagaccatctgaatgggacttatttcttgcacagattgaacggttgattgatcaaagaatagaagcaacagtaagagcaaaagcaatcgctgaattagaaggtttagggagaagttatcaactatatggagaggcatttaaagagtgggaaaaaactccagataacacagcggctcggtctagagtaactgagagatttcgtataattgatgctcaaattgaagcaaatatcccttcgtttcgggtttccggatttgaagtgccacttctattggtttatacccaagcagctaatttgcatctcgctctattaagagattctgttgtttttggagagagatggggattgacgactacaaatgtcaatgatatctataatagacaagttaatagaattggtgaatatagcaatcattgcgtagatacgtataacacagaactagaacgtctagggtttagatctatagcgcagtggagaatatataatcagtttagaagagaactaacactaactgtattagatattgtcgctcttttcccgaactatgacagtagactgtatccgatccaaactttttctcaattgacaagagaaattgttacatccccagtaagcgaattttattatggtgttattaatagtggtaatataaatggtactcttactgaacagcagataaggcgaccacatcttatggacttctttaactccatgatcatgtatacatcagataatagacgggaacattattggtcaggacttgaaatgacggcttattttacaggatttgcaggcgctcaagtgtcattccctttagtcgggactagaggggagtcagctccaccattaactgttagaagtgttaatgatggaatttatagaatattatcggcaccgttttattcagcgccttttctaggcaccattgtattgggaagtcgtggagaaaaatttgattttgcgcttaataatatttcacctccgccatctacaatatacagacatcctggaacagtagattcactagtcagtataccgccacaggataatagcgtaccaccgcacaggggatctagtcatcgattaagtcatgttacaatgcgcgcaagttcccctatattccattggacgcatcgcagcgcaaccactacaaatacaattgatccggagaggattactcaaataccattggtaaaagcacatacacttcagtcaggtactactgttgtaagagggcccgggtttacgggaggagatattcttcgacgaacaagtggaggaccatttgcttatactattgttaatataaatgggcaattaccccaaaggtatcgtgcaagaatacgctatgcctctactacaaatctaagaatttacgtaacggttgcaggtgaacggatttttgctggtcaatttaacaaaacaatggataccggtgacccattaacattccaatcttttagttacgcaactattaatacagcttttacattcccaatgagccagagtagtttcacagtaggtgctgatacttttagttcagggaatgaagtttatatagacagatttgaattgattccagttactgcaacattcgaggcagaatctgatttagaaagagcgcaaaaggcggtgaatgccctgtttacttctacaaaccaactagggctaaaaacagatgtgacggattatcagattgatcaagtgtccaatttagtagaatgtttatcagatgaattttgtctggatgaaaagagagaattgtccgagaaagtcaaacatgcaaagcgacttagtgataagcggaacctacttcaagatccaaacttcacatctatcaatagacaactagaccgtggatggagaggaagtacggatattaccatccaaggaggaaatgacgtattcaaagagaattacgtcacactaccaggtacctttgatgagtgttatccaacgtatttgtatcaaaaaatagatgagtcaaaattaaaagcctatactcgctatgaattaagagggtatattgaagatagtcaagatttagaagtctatttgattcgttacaatgcgaaacatgaaacagtaaatgttcccggtacagggtccttatggccgctttcagtcgaaagcccaatcggaaggtgcggagaaccgaatcgatgtgtgccacatattgaatggaatcctgatttagattgttcgtgtagggatggggagaagtgtgcccatcattcgcatcatttctctctagatattgatgttggatgtacagacctaaatgaggacctaggtgtatgggtgatctttaagattaaaacgcaggatggccatgcaagattaggaaatctagagtttctcgaagagaaaccattgttaggagaagcgttagctcgtgtgaaaagagcggagaaaaaatggagagacaaacgcgaacaattgcagtttgaaacgaatatcgtttacaaagaggcaaaagaatctgtagatgctttattcgtagattctcactataatagattacaagcggatacgaacattacgatgattcatgcggcagataaacgcgttcatcgaatccgagaggcttatcttccggaattatccgttatcccaggtgtaaatgcggacatttttgaagaattagaaggtcttattttcactgcattctccctatatgatgcgagaaatatcattaaaaacggtgatttcaataatggtttatcgtgttggaacgtgaaagggcatgtagatatacaacagaatgatcatcgttctgtcctcgttgtcccggaatgggaatcagaggtatcacaagaagtccgcgtatgtccaggtcgtggctatattcttcgtgtcacagcgtacaaagagggctacggagaaggatgcgtaacgatccatgagatcgaagacaatacagacgaattgaagtttagtaactgcatagaagaggaagtctatccaacggatacaggtaatgattatactgcacaccaaggtacaacaggatgcgcagatgcatgtaattcccgtaatgttggatatgaggatggatatgaaataaatactacagcatctgttaattacaaaccgacttatgaagaagaaatgtatacagatgtacgaagagataatcattgtgaatatgacagaggatatgggaaccatacaccgttaccagctggttatgtaacaaaagaattagagtacttccctgaaacagatacagtatggatagagattggagaaacggaaggaacattcatcgtagatagtgtggaattactcctcatggaggaataa

SEQ ID NO: 30 - DNA, 3507 bp, Artificial Sequence
  Modified Bt toxin
atggagataaataatcagaagcaatgcataccatataattgcttaagtaatcctgaggaagtacttttggatggggagaggatattacctgatatcgatccactcgaagtttctttgtcgcttttgcaatttcttttgaataactttgttccagggggaggctttatttcaggattagttgataaaatatggggggctttgagaccatctgaatgggacttatttcttgcacagattgaacggttgattgatcaaagaatagaagcaacagtaagagcaaaagcaatcgctgaattagaaggtttagggagaagttatcaactatatggagaggcatttaaagagtgggaaaaaactccagataacacagcggctcggtctagagtaactgagagatttcgtataattgatgctcaaattgaagcaaatatcccttcgtttcgggtttccggatttgaagtgccacttctattggtttatacccaagcagctaatttgcatctcgctctattaagagattctgttgtttttggagagagatggggattgacgactacaaatgtcaatgatatctataatagacaagttaatagaattggtgaatatagcaatcattgcgtagatacgtataacacagaactagaacgtctagggtttagatctatagcgcagtggagaatatataatcagtttagaagagaactaacactaactgtattagatattgtcgctcttttcccgaactatgacagtagactgtatccgatccaaactttttctcaattgacaagagaaattgttacatccccagtaagcgaattttattatggtgttattaatagtggtaatataaatggtactcttactgaacagcagataaggcgaccacatcttatggacttctttaactccatgatcatgtatacatcagataatagacgggaacattattggtcaggacttgaaatgacggcttattttacaggatttgcaggcgctcaagtgtcattccctttagtcgggactagaggggagtcagctccaccattaactgttagaagtgttaatgatggaatttatagaatattatcggcaccgttttattcagcgccttttctaggcaccattgtattgggaagtcgtggagaaaaatttgattttgcgcttaataatatttcacctccgccatctacaatatacagacatcctggaacagtagattcactagtcagtataccgccacaggataatagcgtaccaccgcacaggggatctagtcatcgattaagtcatgttacaatgcgcgcaagttcccctatattccattggacgcatcgcagcgcaacccctacaaatacaattgatccggagaggattactcaaataccattggtaaaagcacatacacttcagtcaggtactactgttgtaagagggcccgggtttacgggaggagatattcttcgacgaacaagtggaggaccatttgcttatactattgttaatataaatgggcaattaccccaaaggtatcgtgcaagaatacgctatgcctctactacaaatctaagaatttacgtaacggttgcaggtgaacggatttttgctggtcaatttaacaaaacaatggataccggtgacccattaacattccaatcttttagttacgcaactattaatacagcttttacattcccaatgagccagagtagtttcacagtaggtgctgatacttttagttcagggaatgaagtttatatagacagatttgaattgattccagttactgcaacattcgaggcagaatctgatttagaaagagcgcaaaaggcggtgaatgccctgtttacttctacaaaccaactagggctaaaaacagatgtgacggattatcagattgatcaagtgtccaatttagtagaatgtttatcagatgaattttgtctggatgaaaagagagaattgtccgagaaagtcaaacatgcaaagcgacttagtgataagcggaacctacttcaagatccaaacttcacatctatcaatagacaactagaccgtggatggagaggaagtacggatattaccatccaaggaggaaatgacgtattcaaagagaattacgtcacactaccaggtacctttgatgagtgttatccaacgtatttgtatcaaaaaatagatgagtcaaaattaaaagcctatactcgctatgaattaagagggtatattgaagatagtcaagatttagaagtctatttgattcgttacaatgcgaaacatgaaacagtaaatgttcccggtacagggtccttatggccgctttcagtcgaaagcccaatcggaaggtgcggagaaccgaatcgatgtgtgccacatattgaatggaatcctgatttagattgttcgtgtagggatggggagaagtgtgcccatcattcgcatcatttctctctagatattgatgttggatgtacagacctaaatgaggacctaggtgtatgggtgatctttaagattaaaacgcaggatggccatgcaagattaggaaatctagagtttctcgaagagaaaccattgttaggagaagcgttagctcgtgtgaaaagagcggagaaaaaatggagagacaaacgcgaacaattgcagtttgaaacgaatatcgtttacaaagaggcaaaagaatctgtagatgctttattcgtagattctcactataatagattacaagcggatacgaacattacgatgattcatgcggcagataaacgcgttcatcgaatccgagaggcttatcttccggaattatccgttatcccaggtgtaaatgcggacatttttgaagaattagaaggtcttattttcactgcattctccctatatgatgcgagaaatatcattaaaaacggtgatttcaataatggtttatcgtgttggaacgtgaaagggcatgtagatatacaacagaatgatcatcgttctgtcctcgttgtcccggaatgggaatcagaggtatcacaagaagtccgcgtatgtccaggtcgtggctatattcttcgtgtcacagcgtacaaagagggctacggagaaggatgcgtaacgatccatgagatcgaagacaatacagacgaattgaagtttagtaactgcatagaagaggaagtctatccaacggatacaggtaatgattatactgcacaccaaggtacaacaggatgcgcagatgcatgtaattcccgtaatgttggatatgaggatggatatgaaataaatactacagcatctgttaattacaaaccgacttatgaagaagaaatgtatacagatgtacgaagagataatcattgtgaatatgacagaggatatgggaaccatacaccgttaccagctggttatgtaacaaaagaattagagtacttccctgaaacagatacagtatggatagagattggagaaacggaaggaacattcatcgtagatagtgtggaattactcctcatggaggaataa

SEQ ID NO: 31 - DNA, 3507 bp, Artificial Sequence
  Modified Bt toxin
atggagataaataatcagaagcaatgcataccatataattgcttaagtaatcctgaggaagtacttttggatggggagaggatattacctgatatcgatccactcgaagtttctttgtcgcttttgcaatttcttttgaataactttgttccagggggaggctttatttcaggattagttgataaaatatggggggctttgagaccatctgaatgggacttatttcttgcacagattgaacggttgattgatcaaagaatagaagcaacagtaagagcaaaagcaatcgctgaattagaaggtttagggagaagttatcaactatatggagaggcatttaaagagtgggaaaaaactccagataacacagcggctcggtctagagtaactgagagatttcgtataattgatgctcaaattgaagcaaatatcccttcgtttcgggtttccggatttgaagtgccacttctattggtttatacccaagcagctaatttgcatctcgctctattaagagattctgttgtttttggagagagatggggattgacgactacaaatgtcaatgatatctataatagacaagttaatagaattggtgaatatagcaatcattgcgtagatacgtataacacagaactagaacgtctagggtttagatctatagcgcagtggagaatatataatcagtttagaagagaactaacactaactgtattagatattgtcgctcttttcccgaactatgacagtagactgtatccgatccaaactttttctcaattgacaagagaaattgttacatccccagtaagcgaattttattatggtgttattaatagtggtaatataaatggtactcttactgaacagcagataaggcgaccacatcttatggacttctttaactccatgatcatgtatacatcagataatagacgggaacattattggtcaggacttgaaatgacggcttattttacaggatttgcaggcgctcaagtgtcattccctttagtcgggactagaggggagtcagctccaccattaactgttagaagtgttaatgatggaatttatagaatattatcggcaccgttttattcagcgccttttctaggcaccattgtattgggaagtcgtggagaaaaatttgattttgcgcttaataatatttcacctccgccatctacaatatacagacatcctggaacagtagattcactagtcagtataccgccacaggataatagcgtaccaccgcacaggggatctagtcatcgattaagtcatgttacaatgcgcgcaagttcccctatattccattggacgcatcgcagcgcaaccactacaaatacaattaatccaaatgctattatccaaataccactagtaaaagcacatacacttcagtcaggtactactgttgtaagagggcccgggtttacgggaggagatattcttcgacgaacaagtggaggaccatttgcttatactattgttaatataaatgggcaattaccccaaaggtatcgtgcaagaatacgctatgcctctactacaaatctaagaatttacgtaacggttgcaggtgaacggatttttgctggtcaatttaacaaaacaatggataccggtgacccattaacattccaatcttttagttacgcaactattaatacagcttttacattcccaatgagccagagtagtttcacagtaggtgctgatacttttagttcagggaatgaagtttatatagacagatttgaattgattccagttactgcaacatttgaagcagaatatgatttagaaagagcgcaaaaggcggtgaatgccctgtttacttctacaaaccaactagggctaaaaacagatgtgacggattatcagattgatcaagtgtccaatttagtagaatgtttatcagatgaattttgtctggatgaaaagagagaattgtccgagaaagtcaaacatgcaaagcgacttagtgataagcggaacctacttcaagatccaaacttcacatctatcaatagacaactagaccgtggatggagaggaagtacggatattaccatccaaggaggaaatgacgtattcaaagagaattacgtcacactaccaggtacctttgatgagtgttatccaacgtatttgtatcaaaaaatagatgagtcaaaattaaaagcctatactcgctatgaattaagagggtatattgaagatagtcaagatttagaagtctatttgattcgttacaatgcgaaacatgaaacagtaaatgttcccggtacagggtccttatggccgctttcagtcgaaagcccaatcggaaggtgcggagaaccgaatcgatgtgtgccacatattgaatggaatcctgatttagattgttcgtgtagggatggggagaagtgtgcccatcattcgcatcatttctctctagatattgatgttggatgtacagacctaaatgaggacctaggtgtatgggtgatctttaagattaaaacgcaggatggccatgcaagattaggaaatctagagtttctcgaagagaaaccattgttaggagaagcgttagctcgtgtgaaaagagcggagaaaaaatggagagacaaacgcgaacaattgcagtttgaaacgaatatcgtttacaaagaggcaaaagaatctgtagatgctttattcgtagattctcactataatagattacaagcggatacgaacattacgatgattcatgcggcagataaacgcgttcatcgaatccgagaggcttatcttccggaattatccgttatcccaggtgtaaatgcggacatttttgaagaattagaaggtcttattttcactgcattctccctatatgatgcgagaaatatcattaaaaacggtgatttcaataatggtttatcgtgttggaacgtgaaagggcatgtagatatacaacagaatgatcatcgttctgtcctcgttgtcccggaatgggaatcagaggtatcacaagaagtccgcgtatgtccaggtcgtggctatattcttcgtgtcacagcgtacaaagagggctacggagaaggatgcgtaacgatccatgagatcgaagacaatacagacgaattgaagtttagtaactgcatagaagaggaagtctatccaacggatacaggtaatgattatactgcacaccaaggtacaacaggatgcgcagatgcatgtaattcccgtaatgttggatatgaggatggatatgaaataaatactacagcatctgttaattacaaaccgacttatgaagaagaaatgtatacagatgtacgaagagataatcattgtgaatatgacagaggatatgggaaccatacaccgttaccagctggttatgtaacaaaagaattagagtacttccctgaaacagatacagtatggatagagattggagaaacggaaggaacattcatcgtagatagtgtggaattactcctcatggaggaataa

SEQ ID NO: 32 - DNA, 3507 bp, Artificial Sequence
  Modified Bt toxin
atggagataaataatcagaagcaatgcataccatataattgcttaagtaatcctgaggaagtacttttggatggggagaggatattacctgatatcgatccactcgaagtttctttgtcgcttttgcaatttcttttgaataactttgttccagggggaggctttatttcaggattagttgataaaatatggggggctttgagaccatctgaatgggacttatttcttgcacagattgaacggttgattgatcaaagaatagaagcaacagtaagagcaaaagcaatcgctgaattagaaggtttagggagaagttatcaactatatggagaggcatttaaagagtgggaaaaaactccagataacacagcggctcggtctagagtaactgagagatttcgtataattgatgctcaaattgaagcaaatatcccttcgtttcgggtttccggatttgaagtgccacttctattggtttatacccaagcagctaatttgcatctcgctctattaagagattctgttgtttttggagagagatggggattgacgactacaaatgtcaatgatatctataatagacaagttaatagaattggtgaatatagcaatcattgcgtagatacgtataacacagaactagaacgtctagggtttagatctatagcgcagtggagaatatataatcagtttagaagagaactaacactaactgtattagatattgtcgctcttttcccgaactatgacagtagactgtatccgatccaaactttttctcaattgacaagagaaattgttacatccccagtaagcgaattttattatggtgttattaatagtggtaatataaatggtactcttactgaacagcagataaggcgaccacatcttatggacttctttaactccatgatcatgtatacatcagataatagacgggaacattattggtcaggacttgaaatgacggcttattttacaggatttgcaggcgctcaagtgtcattccctttagtcgggactagaggggagtcagctccaccattaactgttagaagtgttaatgatggaatttatagaatattatcggcaccgttttattcagcgccttttctaggcaccattgtattgggaagtcgtggagaaaaatttgattttgcgcttaataatatttcacctccgccatctacaatatacagacatcctggaacagtagattcactagtcagtataccgccacaggataatagcgtaccaccgcacaggggatctagtcatcgattaagtcatgttacaatgcgcgcaagttcccctatattccattggacgcatcgcagcgcaaccactacaaatacaattgatccggagaggattactcaaataccattggtaaaagcacatacacttcagtcaggtactactgttgtaagagggcccgggtttacgggaggagatattcttcgacgaacaagtggaggaccatttgcttatactattgttaatataaatgggcaattaccccaaaggtatcgtgcaagaatacgctatgcctctactacaaatctaagaatttacgtaacggttgcaggtgaacggatttttgctggtcaatttaacaaaacaatggataccggtgacccattaacattccaatcttttagttacgcaactattaatacagcttttacattcccaatgagccagagtagtttcacagtaggtgctgatacttttagttcagggaatgaagtttatatagacagatttgaattgattccagttactgcaacatttgaagcagaatatgatttagaaagagcgcaaaaggcggtgaatgccctgtttacttctacaaaccaactagggctaaaaacagatgtgacggattatcagattgatcaagtgtccaatttagtagaatgtttatcagatgaattttgtctggatgaaaagagagaattgtccgagaaagtcaaacatgcaaagcgacttagtgataagcggaacctacttcaagatccaaacttcacatctatcaatagacaactagaccgtggatggagaggaagtacggatattaccatccaaggaggaaatgacgtattcaaagagaattacgtcacactaccaggtacctttgatgagtgttatccaacgtatttgtatcaaaaaatagatgagtcaaaattaaaagcctatactcgctatgaattaagagggtatattgaagatagtcaagatttagaagtctatttgattcgttacaatgcgaaacatgaaacagtaaatgttcccggtacagggtccttatggccgctttcagtcgaaagcccaatcggaaggtgcggagaaccgaatcgatgtgtgccacatattgaatggaatcctgatttagattgttcgtgtagggatggggagaagtgtgcccatcattcgcatcatttctctctagatattgatgttggatgtacagacctaaatgaggacctaggtgtatgggtgatctttaagattaaaacgcaggatggccatgcaagattaggaaatctagagtttctcgaagagaaaccattgttaggagaagcgttagctcgtgtgaaaagagcggagaaaaaatggagagacaaacgcgaacaattgcagtttgaaacgaatatcgtttacaaagaggcaaaagaatctgtagatgctttattcgtagattctcactataatagattacaagcggatacgaacattacgatgattcatgcggcagataaacgcgttcatcgaatccgagaggcttatcttccggaattatccgttatcccaggtgtaaatgcggacatttttgaagaattagaaggtcttattttcactgcattctccctatatgatgcgagaaatatcattaaaaacggtgatttcaataatggtttatcgtgttggaacgtgaaagggcatgtagatatacaacagaatgatcatcgttctgtcctcgttgtcccggaatgggaatcagaggtatcacaagaagtccgcgtatgtccaggtcgtggctatattcttcgtgtcacagcgtacaaagagggctacggagaaggatgcgtaacgatccatgagatcgaagacaatacagacgaattgaagtttagtaactgcatagaagaggaagtctatccaacggatacaggtaatgattatactgcacaccaaggtacaacaggatgcgcagatgcatgtaattcccgtaatgttggatatgaggatggatatgaaataaatactacagcatctgttaattacaaaccgacttatgaagaagaaatgtatacagatgtacgaagagataatcattgtgaatatgacagaggatatgggaaccatacaccgttaccagctggttatgtaacaaaagaattagagtacttccctgaaacagatacagtatggatagagattggagaaacggaaggaacattcatcgtagatagtgtggaattactcctcatggaggaataa

SEQ ID NO: 33 - DNA, 3507 bp, Artificial sequence
  Modified Bt toxin
atggagataaataatcagaagcaatgcataccatataattgcttaagtaatcctgaggaagtacttttggatggggagaggatattacctgatatcgatccactcgaagtttctttgtcgcttttgcaatttcttttgaataactttgttccagggggaggctttatttcaggattagttgataaaatatggggggctttgagaccatctgaatgggacttatttcttgcacagattgaacggttgattgatcaaagaatagaagcaacagtaagagcaaaagcaatcgctgaattagaaggtttagggagaagttatcaactatatggagaggcatttaaagagtgggaaaaaactccagataacacagcggctcggtctagagtaactgagagatttcgtataattgatgctcaaattgaagcaaatatcccttcgtttcgggtttccggatttgaagtgccacttctattggtttatacccaagcagctaatttgcatctcgctctattaagagattctgttgtttttggagagagatggggattgacgactacaaatgtcaatgatatctataatagacaagttaatagaattggtgaatatagcaatcattgcgtagatacgtataacacagaactagaacgtctagggtttagatctatagcgcagtggagaatatataatcagtttagaagagaactaacactaactgtattagatattgtcgctcttttcccgaactatgacagtagactgtatccgatccaaactttttctcaattgacaagagaaattgttacatccccagtaagcgaattttattatggtgttattaatagtggtaatataaatggtactcttactgaacagcagataaggcgaccacatcttatggacttctttaactccatgatcatgtatacatcagataatagacgggaacattattggtcaggacttgaaatgacggcttattttacaggatttgcaggcgctcaagtgtcattccctttagtcgggactagaggggagtcagctccaccattaactgttagaagtgttaatgatggaatttatagaatattatcggcaccgttttattcagcgccttttctaggcaccattgtattgggaagtcgtggagaaaaatttgattttgcgcttaataatatttcacctccgccatctacaatatacagacatcctggaacagtagattcactagtcagtataccgccacaggataatagcgtaccaccgcacaggggatctagtcatcgattaagtcatgttacaatgcgcgcaagttcccctatattccattggacgcatcgcagcgcaacccctacaaatacaattgatccggagaggattactcaaataccattggtaaaagcacatacacttcagtcaggtactactgttgtaagagggcccgggtttacgggaggagatattcttcgacgaacaagtggaggaccatttgcttatactattgttaatataaatgggcaattaccccaaaggtatcgtgcaagaatacgctatgcctctactacaaatctaagaatttacgtaacggttgcaggtgaacggatttttgctggtcaatttaacaaaacaatggataccggtgacccattaacattccaatcttttagttacgcaactattaatacagcttttacattcccaatgagccagagtagtttcacagtaggtgctgatacttttagttcagggaatgaagtttatatagacagatttgaattgattccagttactgcaacatttgaagcagaatatgatttagaaagagcgcaaaaggcggtgaatgccctgtttacttctacaaaccaactagggctaaaaacagatgtgacggattatcagattgatcaagtgtccaatttagtagaatgtttatcagatgaattttgtctggatgaaaagagagaattgtccgagaaagtcaaacatgcaaagcgacttagtgataagcggaacctacttcaagatccaaacttcacatctatcaatagacaactagaccgtggatggagaggaagtacggatattaccatccaaggaggaaatgacgtattcaaagagaattacgtcacactaccaggtacctttgatgagtgttatccaacgtatttgtatcaaaaaatagatgagtcaaaattaaaagcctatactcgctatgaattaagagggtatattgaagatagtcaagatttagaagtctatttgattcgttacaatgcgaaacatgaaacagtaaatgttcccggtacagggtccttatggccgctttcagtcgaaagcccaatcggaaggtgcggagaaccgaatcgatgtgtgccacatattgaatggaatcctgatttagattgttcgtgtagggatggggagaagtgtgcccatcattcgcatcatttctctctagatattgatgttggatgtacagacctaaatgaggacctaggtgtatgggtgatctttaagattaaaacgcaggatggccatgcaagattaggaaatctagagtttctcgaagagaaaccattgttaggagaagcgttagctcgtgtgaaaagagcggagaaaaaatggagagacaaacgcgaacaattgcagtttgaaacgaatatcgtttacaaagaggcaaaagaatctgtagatgctttattcgtagattctcactataatagattacaagcggatacgaacattacgatgattcatgcggcagataaacgcgttcatcgaatccgagaggcttatcttccggaattatccgttatcccaggtgtaaatgcggacatttttgaagaattagaaggtcttattttcactgcattctccctatatgatgcgagaaatatcattaaaaacggtgatttcaataatggtttatcgtgttggaacgtgaaagggcatgtagatatacaacagaatgatcatcgttctgtcctcgttgtcccggaatgggaatcagaggtatcacaagaagtccgcgtatgtccaggtcgtggctatattcttcgtgtcacagcgtacaaagagggctacggagaaggatgcgtaacgatccatgagatcgaagacaatacagacgaattgaagtttagtaactgcatagaagaggaagtctatccaacggatacaggtaatgattatactgcacaccaaggtacaacaggatgcgcagatgcatgtaattcccgtaatgttggatatgaggatggatatgaaataaatactacagcatctgttaattacaaaccgacttatgaagaagaaatgtatacagatgtacgaagagataatcattgtgaatatgacagaggatatgggaaccatacaccgttaccagctggttatgtaacaaaagaattagagtacttccctgaaacagatacagtatggatagagattggagaaacggaaggaacattcatcgtagatagtgtggaattactcctcatggaggaataa

SEQ ID NO: 34 - protein, 1169 aa, Artificial Sequence
  BT2-BT2-Cry1Fa-BT29 full-length engineered Cry protein
MEINNQKQCIPYNCLSNPEEVLLDGERILPDIDPLEVSLSLLQFLLNNFVPGGGFISGLVDKIWGALRPSEWDLFLAQIERLIDQRIEATVRAKAIAELEGLGRSYQLYGEAFKEWEKTPDNTAARSRVTERFRIIDAQIEANIPSFRVSGFEVPLLLVYTQAANLHLALLRDSVVFGERWGLTTTNVNDIYNRQVNRIGEYSNHCVDTYNTELERLGFRSIAQWRIYNQFRRELTLTVLDIVALFPNYDSRLYPIQTFSQLTREIVTSPVSEFYYGVINSGNINGTLTEQQIRRPHLMDFFNSMIMYTSDNRREHYWSGLEMTAYFTGFAGAQVSFPLVGTRGESAPPLTVRSVNDGIYRILSAPFYSAPFLGTIVLGSRGEKFDFALNNISPPPSTIYRHPGTVDSLVSIPPQDNSVPPHRGSSHRLSHVTMRASSPIFHWTHRSATTTNTIDPERITQIPLVKAHTLQSGTTVVRGPGFTGGDILRRTSGGPFAYTIVNINGQLPQRYRARIRYASTTNLRIYVTVAGERIFAGQFNKTMDTGDPLTFQSFSYATINTAFTFPMSQSSFTVGADTFSSGNEVYIDRFELIPVTATFEAEYDLEKAQKAVNALFTSSNQIGLKTDVTDYHIDKVSNLVECLSDEFCLDEKRELSEKVKHAKRLCDERNLLQDPNFRGINRQPDRGWRGSTDITIQGGDDVFKENYVTLPGTFDECYPTYLYQKIDESKLKAYTRYELRGYIEDSQDLEIYLIRYNAKHETVNVPGTGSLWPLSAQSPIGKCGEPNRCATHLEWNPDLDCSCRDGEKCAHHSHHFSLDIDVGCTDLNEDLGVWVIFKIKTQDGHARLGNLEFLEEKPLVGEALARVKRAEKKWRDKREKLELETNIVYKEAKKSVDALFVNSQYDRLQADTNIAIIHAADKRVHSIREAYLPELSVIPGVNAAIFEELEGRIFTAYSLYDARNVIKNGDFNNGLSCWNVKGHVDVEEQNNHRSVLVVPEWEAEVSQEVRVCPGRGYILRVTAYKEGYGEGCVTIHEIEDNTDELKFSNCVEEEIYPNNTVTCNDYTATQEEYEGTYTSRNRGYDGAYESNSSVPADYASAYEEKAYTDGRRDNTCESNRGYGDYTPLPAGYVTKELEYFPETDKVWIEIGETEGTFIVDSVELLLMEE

SEQ ID NO: 35 - protein, 1169 aa, Artificial Sequence
  BT2-BT2-BT22-BT29 full-length engineered Cry protein
MEINNQKQCIPYNCLSNPEEVLLDGERILPDIDPLEVSLSLLQFLLNNFVPGGGFISGLVDKIWGALRPSEWDLFLAQIERLIDQRIEATVRAKAIAELEGLGRSYQLYGEAFKEWEKTPDNTAARSRVTERFRIIDAQIEANIPSFRVSGFEVPLLLVYTQAANLHLALLRDSVVFGERWGLTTTNVNDIYNRQVNRIGEYSNHCVDTYNTELERLGFRSIAQWRIYNQFRRELTLTVLDIVALFPNYDSRLYPIQTFSQLTREIVTSPVSEFYYGVINSGNINGTLTEQQIRRPHLMDFFNSMIMYTSDNRREHYWSGLEMTAYFTGFAGAQVSFPLVGTRGESAPPLTVRSVNDGIYRILSAPFYSAPFLGTIVLGSRGEKFDFALNNISPPPSTIYRHPGTVDSLVSIPPQDNSVPPHRGSSHRLSHVTMRASSPIFHWTHRSATTTNTIHSDSITQIPLVKAHTLQSGTTVVKGPGFTGGDILRRTSGGPFAFSNVNLDWNLSQRYRARIRYASTTNLRMYVTIAGERIFAGQFNKTMNTGDPLTFQSFSYATIDTAFTFPTKASSLTVGADTFSSGNEVYVDRFELIPVTATFEAEYDLEKAQKAVNALFTSSNQIGLKTDVTDYHIDKVSNLVECLSDEFCLDEKRELSEKVKHAKRLCDERNLLQDPNFRGINRQPDRGWRGSTDITIQGGDDVFKENYVTLPGTFDECYPTYLYQKIDESKLKAYTRYELRGYIEDSQDLEIYLIRYNAKHETVNVPGTGSLWPLSAQSPIGKCGEPNRCATHLEWNPDLDCSCRDGEKCAHHSHHFSLDIDVGCTDLNEDLGVWVIFKIKTQDGHARLGNLEFLEEKPLVGEALARVKRAEKKWRDKREKLELETNIVYKEAKKSVDALFVNSQYDRLQADTNIAIIHAADKRVHSIREAYLPELSVIPGVNAAIFEELEGRIFTAYSLYDARNVIKNGDFNNGLSCWNVKGHVDVEEQNNHRSVLVVPEWEAEVSQEVRVCPGRGYILRVTAYKEGYGEGCVTIHEIEDNTDELKFSNCVEEEIYPNNTVTCNDYTATQEEYEGTYTSRNRGYDGAYESNSSVPADYASAYEEKAYTDGRRDNTCESNRGYGDYTPLPAGYVTKELEYFPETDKVWIEIGETEGTFIVDSVELLLMEE